European Patent Specification EP 3 224 353 B9, published August 9, 2023. Title: TARGETED ELIMINATION OF BACTERIAL GENES. Applicant: Ramot at Tel-Aviv University Ltd. The sequence listing filed with the application follows.

SEQUENCE LISTING (77 sequences)

SEQ ID NO: 1 - DNA, 30 bp, Artificial Sequence
  Oligonucleotide primer IY344F
accgaagctttgaatatcctccttagttcc

SEQ ID NO: 2 - DNA, 50 bp, Artificial Sequence
  Oligonucleotide primer IY344R
cgccaagcttacggggcaacctcatgtcaagtgtaggctggagctgcttc

SEQ ID NO: 3 - DNA, 20 bp, Artificial Sequence
  Oligonucleotide primer IY246F
atggaattgcccaatattat

SEQ ID NO: 4 - DNA, 20 bp, Artificial Sequence
  Oligonucleotide primer IY246R
tcagcgcagcttgtcggcca

SEQ ID NO: 5 - DNA, 35 bp, Artificial Sequence
  Oligonucleotide primer IY247F
gaactaaatcaggcacttgagcatcaagattggtg

SEQ ID NO: 6 - DNA, 35 bp, Artificial Sequence
  Oligonucleotide primer IY247R
caccaatcttgatgctcaagtgcctgatttagttc

SEQ ID NO: 7 - DNA, 25 bp, Artificial Sequence
  Oligonucleotide primer IY346F
atggttaaaaaatcactgcgccagt

SEQ ID NO: 8 - DNA, 20 bp, Artificial Sequence
  Oligonucleotide primer IY346R
ttacaaaccgtcggtgacga

SEQ ID NO: 9 - DNA, 20 bp, Artificial Sequence
  Oligonucleotide primer IY142Fb
cacacggtcacactgcttcc

SEQ ID NO: 10 - DNA, 20 bp, Artificial Sequence
  Oligonucleotide primer MG110R
cgatgcccttgagagccttc

SEQ ID NO: 11 - DNA, 20 bp, Artificial Sequence
  Oligonucleotide primer MG17F
ataagtcggacaccatggca

SEQ ID NO: 12 - DNA, 70 bp, Artificial Sequence
  Oligonucleotide primer IY80F
aatagcccgctgatatcatcgataatactaaaaaaacagggaggctattagtgtaggctggagctgcttc

SEQ ID NO: 13 - DNA, 70 bp, Artificial Sequence
  Oligonucleotide primer IY80R
accttaatgtaacatttccttattattaaagatcagctaattctttgttttgaatatcctccttagttcc

SEQ ID NO: 14 - DNA, 73 bp, Artificial Sequence
  Oligonucleotide primer IY333F
atgcgtaatgtgtgtattgccgttgctgtctttgccgcacttgcggtgacccggaatgaaattaatacgactc

SEQ ID NO: 15 - DNA, 70 bp, Artificial Sequence
  Oligonucleotide primer IY333R
aacctgtcgcactccagagaagcacaaagcctcgcaatccagtgcaaagctcacagtggagccaaagata

SEQ ID NO: 16 - DNA, 70 bp, Artificial Sequence
  Oligonucleotide primer IY347F
ggccagctaaatcgatgggatgtggcttgctatctttggctccactgtgagggatgtgctgcaaggcgat

SEQ ID NO: 17 - DNA, 70 bp, Artificial Sequence
  Oligonucleotide primer IY347R
aacctgtcgcactccagagaagcacaaagcctcgcaatccagtgcaaagcacggggcaacctcatgtcaa

SEQ ID NO: 18 - DNA, 75 bp, Artificial Sequence
  Oligonucleotide primer IY309F
accctcaagagaaaatgtaaaagctgtctttcgctgctgagggtgacgatcccgcgatccgtcagcctgcagttc

SEQ ID NO: 19 - DNA, 75 bp, Artificial Sequence
  Oligonucleotide primer IY309R
ccgaaggtgagccagtgtgaaagctgtctttcgctgctgagggtgacgatcccgctgtaggctggagctgcttcg

SEQ ID NO: 20 - DNA, 75 bp, Artificial Sequence
  Oligonucleotide primer IY340Fa
accctcaagagaaaatgtaaaagctgagcaccgcattagccgctgcattgatgctgatccgtcagcctgcagttc

SEQ ID NO: 21 - DNA, 75 bp, Artificial Sequence
  Oligonucleotide primer IY340Fb
accctcaagagaaaatgtaaaagctgattgctcacgttggcggcccggctagcgtgatccgtcagcctgcagttc

SEQ ID NO: 22 - DNA, 75 bp, Artificial Sequence
  Oligonucleotide primer IY340Ra
ccgaaggtgagccagtgtgagtacgtccgccgtttgcgcatacagcggcacactttgtaggctggagctgcttcg

SEQ ID NO: 23 - DNA, 75 bp, Artificial Sequence
  Oligonucleotide primer IY340Rb
ccgaaggtgagccagtgtgaaccgccagcgcgaccggcaggttgatctcctgctttgtaggctggagctgcttcg

SEQ ID NO: 24 - DNA, 70 bp, Artificial Sequence
  Oligonucleotide primer IY260F
tggctctttgcggcacccatcgttcgtaatgttccgtggcaccgaggacaaccctcaagagaaaatgtaa

SEQ ID NO: 25 - DNA, 70 bp, Artificial Sequence
  Oligonucleotide primer IY260R
ccaaccttcttaaacataaagtgtctccttataaacgcagaaaggcccacccgaaggtgagccagtgtga

SEQ ID NO: 26 - DNA, 19 bp, Artificial Sequence
  Oligonucleotide primer RK41F
ggaattacttcgcttcgcc

SEQ ID NO: 27 - DNA, 56 bp, Artificial Sequence
  Oligonucleotide primer RK41R
cctccttatctccctatagtgagtcgtattaatttcattccggggatccgtcgacc

SEQ ID NO: 28 - DNA, 70 bp, Artificial Sequence
  Oligonucleotide primer RK42F
aaacgcgtttctttggcttaaaaagggaatgtgggttacacgaagggtaatgtaggctggagctgcttcg

SEQ ID NO: 29 - DNA, 70 bp, Artificial Sequence
  Oligonucleotide primer RK42R
ggattttccccagtaatggcatatatatttaaaaggttccattaatagcccctccttatctccctatagt

SEQ ID NO: 30 - DNA, 20 bp, Artificial Sequence
  Oligonucleotide primer RK43F
gcagcattacacgtcttgag

SEQ ID NO: 31 - DNA, 55 bp, Artificial Sequence
  Oligonucleotide primer RK43R
ctccttatctccctatagtgagtcgtattaatttctgaatatcctccttagttcc

SEQ ID NO: 32 - DNA, 70 bp, Artificial Sequence
  Oligonucleotide primer RK44F
ttcgggaatgattgttatcaatgacgataataagaccaataacggtttatgtgtaggctggagctgcttc

SEQ ID NO: 33 - DNA, 70 bp, Artificial Sequence
  Oligonucleotide primer RK44R
cgcgggcgtacagggatccagttatcaataagcaaattcatttgttctccctccttatctccctatagtg

SEQ ID NO: 34 - DNA, 30 bp, Artificial Sequence
  Oligonucleotide primer RK29R
gactctcgaggccactgatctctactgcag

SEQ ID NO: 35 - DNA, 30 bp, Artificial Sequence
  Oligonucleotide primer RK33R
gactctcgaggcaacagcagcaacatcaag

SEQ ID NO: 36 - DNA, 48502 bp, Bacteriophage lambda
gggcggcgacctcgcgggttttcgctatttatgaaaattttccggtttaaggcgtttccgttcttcttcgtcataacttaatgtttttatttaaaataccctctgaaaagaaaggaaacgacaggtgctgaaagcgaggctttttggcctctgtcgtttcctttctctgtttttgtccgtggaatgaacaatggaagtcaacaaaaagcagctggctgacattttcggtgcgagtatccgtaccattcagaactggcaggaacagggaatgcccgttctgcgaggcggtggcaagggtaatgaggtgctttatgactctgccgccgtcataaaatggtatgccgaaagggatgctgaaattgagaacgaaaagctgcgccgggaggttgaagaactgcggcaggccagcgaggcagatctccagccaggaactattgagtacgaacgccatcgacttacgcgtgcgcaggccgacgcacaggaactgaagaatgccagagactccgctgaagtggtggaaaccgcattctgtactttcgtgctgtcgcggatcgcaggtgaaattgccagtattctcgacgggctccccctgtcggtgcagcggcgttttccggaactggaaaaccgacatgttgatttcctgaaacgggatatcatcaaagccatgaacaaagcagccgcgctggatgaactgataccggggttgctgagtgaatatatcgaacagtcaggttaacaggctgcggcattttgtccgcgccgggcttcgctcactgttcaggccggagccacagaccgccgttgaatgggcggatgctaattactatctcccgaaagaatccgcataccaggaagggcgctgggaaacactgccctttcagcgggccatcatgaatgcgatgggcagcgactacatccgtgaggtgaatgtggtgaagtctgcccgtgtcggttattccaaaatgctgctgggtgtttatgcctactttatagagcataagcagcgcaacacccttatctggttgccgacggatggtgatgccgagaactttatgaaaacccacgttgagccgactattcgtgatattccgtcgctgctggcgctggccccgtggtatggcaaaaagcaccgggataacacgctcaccatgaagcgtttcactaatgggcgtggcttctggtgcctgggcggtaaagcggcaaaaaactaccgtgaaaagtcggtggatgtggcgggttatgatgaacttgctgcttttgatgatgatattgaacaggaaggctctccgacgttcctgggtgacaagcgtattgaaggctcggtctggccaaagtccatccgtggctccacgccaaaagtgagaggcacctgtcagattgagcgtgcagccagtgaatccccgcattttatgcgttttcatgttgcctgcccgcattgcggggaggagcagtatcttaaatttggcgacaaagagacgccgtttggcctcaaatggacgccggatgacccctccagcgtgttttatctctgcgagcataatgcctgcgtcatccgccagcaggagctggactttactgatgcccgttatatctgcgaaaagaccgggatctggacccgtgatggcattctctggttttcgtcatccggtgaagagattgagccacctgacagtgtgacctttcacatctggacagcgtacagcccgttcaccacctgggtgcagattgtcaaagactggatgaaaacgaaaggggatacgggaaaacgtaaaaccttcgtaaacaccacgctcggtgagacgtgggaggcgaaaattggcgaacgtccggatgctgaagtgatggcagagcggaaagagcattattcagcgcccgttcctgaccgtgtggcttacctgaccgccggtatcgactcccagctggaccgctacgaaatgcgcgtatggggatgggggccgggtgaggaaagctggctgattgaccggcagattattatgggccgccacgacgatgaacagacgctgctgcgtgtggatgaggccatcaataaaacctatacccgccggaatggtgcagaaatgtcgatatcccgtatctgctgggatactggcgggattgacccgaccattgtgtatgaacgctcgaaaaaacatgggctgttccgggtgatccccattaaaggggcatccgtctacggaaagccggtggccagcatgccacgtaagcgaaacaaaaacggggtttaccttaccgaaatcggtacggataccgcgaaagagcagatttataaccgcttcacactgacgccggaaggggatgaaccgcttcccggtgccgttcacttcccgaataacccggatatttttgatctgaccgaagcgcagcagctgactgctgaagagcaggtcgaaaaatgggtggatggcaggaaaaaaatactgtgggacagcaaaaagcgacgcaatgaggcactcgactgcttcgtttatgcgctggcggcgctgcgcatcagtatttcccgctggcagctggatctcagtgcgctgctggcgagcctgcaggaagaggatggtgcagcaaccaacaagaaaacactggcagattacgcccgtgccttatccggagaggatgaatgacgcgacaggaagaacttgccgctgcccgtgcggcactgcatgacctgatgacaggtaaacgggtggcaacagtacagaaagacggacgaagggtggagtttacggccacttccgtgtctgacctgaaaaaatatattgcagagctggaagtgcagaccggcatgacacagcgacgcaggggacctgcaggattttatgtatgaaaacgcccaccattcccacccttctggggccggacggcatgacatcgctgcgcgaatatgccggttatcacggcggtggcagcggatttggagggcagttgcggtcgtggaacccaccgagtgaaagtgtggatgcagccctgttgcccaactttacccgtggcaatgcccgcgcagacgatctggtacgcaataacggctatgccgccaacgccatccagctgcatcaggatcatatcgtcgggtcttttttccggctcagtcatcgcccaagctggcgctatctgggcatcggggaggaagaagcccgtgccttttcccgcgaggttgaagcggcatggaaagagtttgccgaggatgactgctgctgcattgacgttgagcgaaaacgcacgtttaccatgatgattcgggaaggtgtggccatgcacgcctttaacggtgaactgttcgttcaggccacctgggataccagttcgtcgcggcttttccggacacagttccggatggtcagcccgaagcgcatcagcaacccgaacaataccggcgacagccggaactgccgtgccggtgtgcagattaatgacagcggtgcggcgctgggatattacgtcagcgaggacgggtatcctggctggatgccgcagaaatggacatggataccccgtgagttacccggcgggcgcgcctcgttcattcacgtttttgaacccgtggaggacgggcagactcgcggtgcaaatgtgttttacagcgtgatggagcagatgaagatgctcgacacgctgcagaacacgcagctgcagagcgccattgtgaaggcgatgtatgccgccaccattgagagtgagctggatacgcagtcagcgatggattttattctgggcgcgaacagtcaggagcagcgggaaaggctgaccggctggattggtgaaattgccgcgtattacgccgcagcgccggtccggctgggaggcgcaaaagtaccgcacctgatgccgggtgactcactgaacctgcagacggctcaggatacggataacggctactccgtgtttgagcagtcactgctgcggtatatcgctgccgggctgggtgtctcgtatgagcagctttcccggaattacgcccagatgagctactccacggcacgggccagtgcgaacgagtcgtgggcgtactttatggggcggcgaaaattcgtcgcatcccgtcaggcgagccagatgtttctgtgctggctggaagaggccatcgttcgccgcgtggtgacgttaccttcaaaagcgcgcttcagttttcaggaagcccgcagtgcctgggggaactgcgactggataggctccggtcgtatggccatcgatggtctgaaagaagttcaggaagcggtgatgctgatagaagccggactgagtacctacgagaaagagtgcgcaaaacgcggtgacgactatcaggaaatttttgcccagcaggtccgtgaaacgatggagcgccgtgcagccggtcttaaaccgcccgcctgggcggctgcagcatttgaatccgggctgcgacaatcaacagaggaggagaagagtgacagcagagctgcgtaatctcccgcatattgccagcatggcctttaatgagccgctgatgcttgaacccgcctatgcgcgggttttcttttgtgcgcttgcaggccagcttgggatcagcagcctgacggatgcggtgtccggcgacagcctgactgcccaggaggcactcgcgacgctggcattatccggtgatgatgacggaccacgacaggcccgcagttatcaggtcatgaacggcatcgccgtgctgccggtgtccggcacgctggtcagccggacgcgggcgctgcagccgtactcggggatgaccggttacaacggcattatcgcccgtctgcaacaggctgccagcgatccgatggtggacggcattctgctcgatatggacacgcccggcgggatggtggcgggggcatttgactgcgctgacatcatcgcccgtgtgcgtgacataaaaccggtatgggcgcttgccaacgacatgaactgcagtgcaggtcagttgcttgccagtgccgcctcccggcgtctggtcacgcagaccgcccggacaggctccatcggcgtcatgatggctcacagtaattacggtgctgcgctggagaaacagggtgtggaaatcacgctgatttacagcggcagccataaggtggatggcaacccctacagccatcttccggatgacgtccgggagacactgcagtcccggatggacgcaacccgccagatgtttgcgcagaaggtgtcggcatataccggcctgtccgtgcaggttgtgctggataccgaggctgcagtgtacagcggtcaggaggccattgatgccggactggctgatgaacttgttaacagcaccgatgcgatcaccgtcatgcgtgatgcactggatgcacgtaaatcccgtctctcaggagggcgaatgaccaaagagactcaatcaacaactgtttcagccactgcttcgcaggctgacgttactgacgtggtgccagcgacggagggcgagaacgccagcgcggcgcagccggacgtgaacgcgcagatcaccgcagcggttgcggcagaaaacagccgcattatggggatcctcaactgtgaggaggctcacggacgcgaagaacaggcacgcgtgctggcagaaacccccggtatgaccgtgaaaacggcccgccgcattctggccgcagcaccacagagtgcacaggcgcgcagtgacactgcgctggatcgtctgatgcagggggcaccggcaccgctggctgcaggtaacccggcatctgatgccgttaacgatttgctgaacacaccagtgtaagggatgtttatgacgagcaaagaaacctttacccattaccagccgcagggcaacagtgacccggctcataccgcaaccgcgcccggcggattgagtgcgaaagcgcctgcaatgaccccgctgatgctggacacctccagccgtaagctggttgcgtgggatggcaccaccgacggtgctgccgttggcattcttgcggttgctgctgaccagaccagcaccacgctgacgttctacaagtccggcacgttccgttatgaggatgtgctctggccggaggctgccagcgacgagacgaaaaaacggaccgcgtttgccggaacggcaatcagcatcgtttaactttacccttcatcactaaaggccgcctgtgcggctttttttacgggatttttttatgtcgatgtacacaaccgcccaactgctggcggcaaatgagcagaaatttaagtttgatccgctgtttctgcgtctctttttccgtgagagctatcccttcaccacggagaaagtctatctctcacaaattccgggactggtaaacatggcgctgtacgtttcgccgattgtttccggtgaggttatccgttcccgtggcggctccacctctgaatttacgccgggatatgtcaagccgaagcatgaagtgaatccgcagatgaccctgcgtcgcctgccggatgaagatccgcagaatctggcggacccggcttaccgccgccgtcgcatcatcatgcagaacatgcgtgacgaagagctggccattgctcaggtcgaagagatgcaggcagtttctgccgtgcttaagggcaaatacaccatgaccggtgaagccttcgatccggttgaggtggatatgggccgcagtgaggagaataacatcacgcagtccggcggcacggagtggagcaagcgtgacaagtccacgtatgacccgaccgacgatatcgaagcctacgcgctgaacgccagcggtgtggtgaatatcatcgtgttcgatccgaaaggctgggcgctgttccgttccttcaaagccgtcaaggagaagctggatacccgtcgtggctctaattccgagctggagacagcggtgaaagacctgggcaaagcggtgtcctataaggggatgtatggcgatgtggccatcgtcgtgtattccggacagtacgtggaaaacggcgtcaaaaagaacttcctgccggacaacacgatggtgctggggaacactcaggcacgcggtctgcgcacctatggctgcattcaggatgcggacgcacagcgcgaaggcattaacgcctctgcccgttacccgaaaaactgggtgaccaccggcgatccggcgcgtgagttcaccatgattcagtcagcaccgctgatgctgctggctgaccctgatgagttcgtgtccgtacaactggcgtaatcatggcccttcggggccattgtttctctgtggaggagtccatgacgaaagatgaactgattgcccgtctccgctcgctgggtgaacaactgaaccgtgatgtcagcctgacggggacgaaagaagaactggcgctccgtgtggcagagctgaaagaggagcttgatgacacggatgaaactgccggtcaggacacccctctcagccgggaaaatgtgctgaccggacatgaaaatgaggtgggatcagcgcagccggataccgtgattctggatacgtctgaactggtcacggtcgtggcactggtgaagctgcatactgatgcacttcacgccacgcgggatgaacctgtggcatttgtgctgccgggaacggcgtttcgtgtctctgccggtgtggcagccgaaatgacagagcgcggcctggccagaatgcaataacgggaggcgctgtggctgatttcgataacctgttcgatgctgccattgcccgcgccgatgaaacgatacgcgggtacatgggaacgtcagccaccattacatccggtgagcagtcaggtgcggtgatacgtggtgtttttgatgaccctgaaaatatcagctatgccggacagggcgtgcgcgttgaaggctccagcccgtccctgtttgtccggactgatgaggtgcggcagctgcggcgtggagacacgctgaccatcggtgaggaaaatttctgggtagatcgggtttcgccggatgatggcggaagttgtcatctctggcttggacggggcgtaccgcctgccgttaaccgtcgccgctgaaagggggatgtatggccataaaaggtcttgagcaggccgttgaaaacctcagccgtatcagcaaaacggcggtgcctggtgccgccgcaatggccattaaccgcgttgcttcatccgcgatatcgcagtcggcgtcacaggttgcccgtgagacaaaggtacgccggaaactggtaaaggaaagggccaggctgaaaagggccacggtcaaaaatccgcaggccagaatcaaagttaaccggggggatttgcccgtaatcaagctgggtaatgcgcgggttgtcctttcgcgccgcaggcgtcgtaaaaaggggcagcgttcatccctgaaaggtggcggcagcgtgcttgtggtgggtaaccgtcgtattcccggcgcgtttattcagcaactgaaaaatggccggtggcatgtcatgcagcgtgtggctgggaaaaaccgttaccccattgatgtggtgaaaatcccgatggcggtgccgctgaccacggcgtttaaacaaaatattgagcggatacggcgtgaacgtcttccgaaagagctgggctatgcgctgcagcatcaactgaggatggtaataaagcgatgaaacatactgaactccgtgcagccgtactggatgcactggagaagcatgacaccggggcgacgttttttgatggtcgccccgctgtttttgatgaggcggattttccggcagttgccgtttatctcaccggcgctgaatacacgggcgaagagctggacagcgatacctggcaggcggagctgcatatcgaagttttcctgcctgctcaggtgccggattcagagctggatgcgtggatggagtcccggatttatccggtgatgagcgatatcccggcactgtcagatttgatcaccagtatggtggccagcggctatgactaccggcgcgacgatgatgcgggcttgtggagttcagccgatctgacttatgtcattacctatgaaatgtgaggacgctatgcctgtaccaaatcctacaatgccggtgaaaggtgccgggaccaccctgtgggtttataaggggagcggtgacccttacgcgaatccgctttcagacgttgactggtcgcgtctggcaaaagttaaagacctgacgcccggcgaactgaccgctgagtcctatgacgacagctatctcgatgatgaagatgcagactggactgcgaccgggcaggggcagaaatctgccggagataccagcttcacgctggcgtggatgcccggagagcaggggcagcaggcgctgctggcgtggtttaatgaaggcgatacccgtgcctataaaatccgcttcccgaacggcacggtcgatgtgttccgtggctgggtcagcagtatcggtaaggcggtgacggcgaaggaagtgatcacccgcacggtgaaagtcaccaatgtgggacgtccgtcgatggcagaagatcgcagcacggtaacagcggcaaccggcatgaccgtgacgcctgccagcacctcggtggtgaaagggcagagcaccacgctgaccgtggccttccagccggagggcgtaaccgacaagagctttcgtgcggtgtctgcggataaaacaaaagccaccgtgtcggtcagtggtatgaccatcaccgtgaacggcgttgctgcaggcaaggtcaacattccggttgtatccggtaatggtgagtttgctgcggttgcagaaattaccgtcaccgccagttaatccggagagtcagcgatgttcctgaaaaccgaatcatttgaacataacggtgtgaccgtcacgctttctgaactgtcagccctgcagcgcattgagcatctcgccctgatgaaacggcaggcagaacaggcggagtcagacagcaaccggaagtttactgtggaagacgccatcagaaccggcgcgtttctggtggcgatgtccctgtggcataaccatccgcagaagacgcagatgccgtccatgaatgaagccgttaaacagattgagcaggaagtgcttaccacctggcccacggaggcaatttctcatgctgaaaacgtggtgtaccggctgtctggtatgtatgagtttgtggtgaataatgcccctgaacagacagaggacgccgggcccgcagagcctgtttctgcgggaaagtgttcgacggtgagctgagttttgccctgaaactggcgcgtgagatggggcgacccgactggcgtgccatgcttgccgggatgtcatccacggagtatgccgactggcaccgcttttacagtacccattattttcatgatgttctgctggatatgcacttttccgggctgacgtacaccgtgctcagcctgtttttcagcgatccggatatgcatccgctggatttcagtctgctgaaccggcgcgaggctgacgaagagcctgaagatgatgtgctgatgcagaaagcggcagggcttgccggaggtgtccgctttggcccggacgggaatgaagttatccccgcttccccggatgtggcggacatgacggaggatgacgtaatgctgatgacagtatcagaagggatcgcaggaggagtccggtatggctgaaccggtaggcgatctggtcgttgatttgagtctggatgcggccagatttgacgagcagatggccagagtcaggcgtcatttttctggtacggaaagtgatgcgaaaaaaacagcggcagtcgttgaacagtcgctgagccgacaggcgctggctgcacagaaagcggggatttccgtcgggcagtataaagccgccatgcgtatgctgcctgcacagttcaccgacgtggccacgcagcttgcaggcgggcaaagtccgtggctgatcctgctgcaacagggggggcaggtgaaggactccttcggcgggatgatccccatgttcagggggcttgccggtgcgatcaccctgccgatggtgggggccacctcgctggcggtggcgaccggtgcgctggcgtatgcctggtatcagggcaactcaaccctgtccgatttcaacaaaacgctggtcctttccggcaatcaggcgggactgacggcagatcgtatgctggtcctgtccagagccgggcaggcggcagggctgacgtttaaccagaccagcgagtcactcagcgcactggttaaggcgggggtaagcggtgaggctcagattgcgtccatcagccagagtgtggcgcgtttctcctctgcatccggcgtggaggtggacaaggtcgctgaagccttcgggaagctgaccacagacccgacgtcggggctgacggcgatggctcgccagttccataacgtgtcggcggagcagattgcgtatgttgctcagttgcagcgttccggcgatgaagccggggcattgcaggcggcgaacgaggccgcaacgaaagggtttgatgaccagacccgccgcctgaaagagaacatgggcacgctggagacctgggcagacaggactgcgcgggcattcaaatccatgtgggatgcggtgctggatattggtcgtcctgataccgcgcaggagatgctgattaaggcagaggctgcgtataagaaagcagacgacatctggaatctgcgcaaggatgattattttgttaacgatgaagcgcgggcgcgttactgggatgatcgtgaaaaggcccgtcttgcgcttgaagccgcccgaaagaaggctgagcagcagactcaacaggacaaaaatgcgcagcagcagagcgataccgaagcgtcacggctgaaatataccgaagaggcgcagaaggcttacgaacggctgcagacgccgctggagaaatataccgcccgtcaggaagaactgaacaaggcactgaaagacgggaaaatcctgcaggcggattacaacacgctgatggcggcggcgaaaaaggattatgaagcgacgctgaaaaagccgaaacagtccagcgtgaaggtgtctgcgggcgatcgtcaggaagacagtgctcatgctgccctgctgacgcttcaggcagaactccggacgctggagaagcatgccggagcaaatgagaaaatcagccagcagcgccgggatttgtggaaggcggagagtcagttcgcggtactggaggaggcggcgcaacgtcgccagctgtctgcacaggagaaatccctgctggcgcataaagatgagacgctggagtacaaacgccagctggctgcacttggcgacaaggttacgtatcaggagcgcctgaacgcgctggcgcagcaggcggataaattcgcacagcagcaacgggcaaaacgggccgccattgatgcgaaaagccgggggctgactgaccggcaggcagaacgggaagccacggaacagcgcctgaaggaacagtatggcgataatccgctggcgctgaataacgtcatgtcagagcagaaaaagacctgggcggctgaagaccagcttcgcgggaactggatggcaggcctgaagtccggctggagtgagtgggaagagagcgccacggacagtatgtcgcaggtaaaaagtgcagccacgcagacctttgatggtattgcacagaatatggcggcgatgctgaccggcagtgagcagaactggcgcagcttcacccgttccgtgctgtccatgatgacagaaattctgcttaagcaggcaatggtggggattgtcgggagtatcggcagcgccattggcggggctgttggtggcggcgcatccgcgtcaggcggtacagccattcaggccgctgcggcgaaattccattttgcaaccggaggatttacgggaaccggcggcaaatatgagccagcggggattgttcaccgtggtgagtttgtcttcacgaaggaggcaaccagccggattggcgtggggaatctttaccggctgatgcgcggctatgccaccggcggttatgtcggtacaccgggcagcatggcagacagccggtcgcaggcgtccgggacgtttgagcagaataaccatgtggtgattaacaacgacggcacgaacgggcagataggtccggctgctctgaaggcggtgtatgacatggcccgcaagggtgcccgtgatgaaattcagacacagatgcgtgatggtggcctgttctccggaggtggacgatgaagaccttccgctggaaagtgaaacccggtatggatgtggcttcggtcccttctgtaagaaaggtgcgctttggtgatggctattctcagcgagcgcctgccgggctgaatgccaacctgaaaacgtacagcgtgacgctttctgtcccccgtgaggaggccacggtactggagtcgtttctggaagagcacgggggctggaaatcctttctgtggacgccgccttatgagtggcggcagataaaggtgacctgcgcaaaatggtcgtcgcgggtcagtatgctgcgtgttgagttcagcgcagagtttgaacaggtggtgaactgatgcaggatatccggcaggaaacactgaatgaatgcacccgtgcggagcagtcggccagcgtggtgctctgggaaatcgacctgacagaggtcggtggagaacgttattttttctgtaatgagcagaacgaaaaaggtgagccggtcacctggcaggggcgacagtatcagccgtatcccattcaggggagcggttttgaactgaatggcaaaggcaccagtacgcgccccacgctgacggtttctaacctgtacggtatggtcaccgggatggcggaagatatgcagagtctggtcggcggaacggtggtccggcgtaaggtttacgcccgttttctggatgcggtgaacttcgtcaacggaaacagttacgccgatccggagcaggaggtgatcagccgctggcgcattgagcagtgcagcgaactgagcgcggtgagtgcctcctttgtactgtccacgccgacggaaacggatggcgctgtttttccgggacgtatcatgctggccaacacctgcacctggacctatcgcggtgacgagtgcggttatagcggtccggctgtcgcggatgaatatgaccagccaacgtccgatatcacgaaggataaatgcagcaaatgcctgagcggttgtaagttccgcaataacgtcggcaactttggcggcttcctttccattaacaaactttcgcagtaaatcccatgacacagacagaatcagcgattctggcgcacgcccggcgatgtgcgccagcggagtcgtgcggcttcgtggtaagcacgccggagggggaaagatatttcccctgcgtgaatatctccggtgagccggaggctatttccgtatgtcgccggaagactggctgcaggcagaaatgcagggtgagattgtggcgctggtccacagccaccccggtggtctgccctggctgagtgaggccgaccggcggctgcaggtgcagagtgatttgccgtggtggctggtctgccgggggacgattcataagttccgctgtgtgccgcatctcaccgggcggcgctttgagcacggtgtgacggactgttacacactgttccgggatgcttatcatctggcggggattgagatgccggactttcatcgtgaggatgactggtggcgtaacggccagaatctctatctggataatctggaggcgacggggctgtatcaggtgccgttgtcagcggcacagccgggcgatgtgctgctgtgctgttttggttcatcagtgccgaatcacgccgcaatttactgcggcgacggcgagctgctgcaccatattcctgaacaactgagcaaacgagagaggtacaccgacaaatggcagcgacgcacacactccctctggcgtcaccgggcatggcgcgcatctgcctttacggggatttacaacgatttggtcgccgcatcgaccttcgtgtgaaaacgggggctgaagccatccgggcactggccacacagctcccggcgtttcgtcagaaactgagcgacggctggtatcaggtacggattgccgggcgggacgtcagcacgtccgggttaacggcgcagttacatgagactctgcctgatggcgctgtaattcatattgttcccagagtcgccggggccaagtcaggtggcgtattccagattgtcctgggggctgccgccattgccggatcattctttaccgccggagccacccttgcagcatggggggcagccattggggccggtggtatgaccggcatcctgttttctctcggtgccagtatggtgctcggtggtgtggcgcagatgctggcaccgaaagccagaactccccgtatacagacaacggataacggtaagcagaacacctatttctcctcactggataacatggttgcccagggcaatgttctgcctgttctgtacggggaaatgcgcgtggggtcacgcgtggtttctcaggagatcagcacggcagacgaaggggacggtggtcaggttgtggtgattggtcgctgatgcaaaatgttttatgtgaaaccgcctgcgggcggttttgtcatttatggagcgtgaggaatgggtaaaggaagcagtaaggggcataccccgcgcgaagcgaaggacaacctgaagtccacgcagttgctgagtgtgatcgatgccatcagcgaagggccgattgaaggtccggtggatggcttaaaaagcgtgctgctgaacagtacgccggtgctggacactgaggggaataccaacatatccggtgtcacggtggtgttccgggctggtgagcaggagcagactccgccggagggatttgaatcctccggctccgagacggtgctgggtacggaagtgaaatatgacacgccgatcacccgcaccattacgtctgcaaacatcgaccgtctgcgctttaccttcggtgtacaggcactggtggaaaccacctcaaagggtgacaggaatccgtcggaagtccgcctgctggttcagatacaacgtaacggtggctgggtgacggaaaaagacatcaccattaagggcaaaaccacctcgcagtatctggcctcggtggtgatgggtaacctgccgccgcgcccgtttaatatccggatgcgcaggatgacgccggacagcaccacagaccagctgcagaacaaaacgctctggtcgtcatacactgaaatcatcgatgtgaaacagtgctacccgaacacggcactggtcggcgtgcaggtggactcggagcagttcggcagccagcaggtgagccgtaattatcatctgcgcgggcgtattctgcaggtgccgtcgaactataacccgcagacgcggcaatacagcggtatctgggacggaacgtttaaaccggcatacagcaacaacatggcctggtgtctgtgggatatgctgacccatccgcgctacggcatggggaaacgtcttggtgcggcggatgtggataaatgggcgctgtatgtcatcggccagtactgcgaccagtcagtgccggacggctttggcggcacggagccgcgcatcacctgtaatgcgtacctgaccacacagcgtaaggcgtgggatgtgctcagcgatttctgctcggcgatgcgctgtatgccggtatggaacgggcagacgctgacgttcgtgcaggaccgaccgtcggataagacgtggacctataaccgcagtaatgtggtgatgccggatgatggcgcgccgttccgctacagcttcagcgccctgaaggaccgccataatgccgttgaggtgaactggattgacccgaacaacggctgggagacggcgacagagcttgttgaagatacgcaggccattgcccgttacggtcgtaatgttacgaagatggatgcctttggctgtaccagccgggggcaggcacaccgcgccgggctgtggctgattaaaacagaactgctggaaacgcagaccgtggatttcagcgtcggcgcagaagggcttcgccatgtaccgggcgatgttattgaaatctgcgatgatgactatgccggtatcagcaccggtggtcgtgtgctggcggtgaacagccagacccggacgctgacgctcgaccgtgaaatcacgctgccatcctccggtaccgcgctgataagcctggttgacggaagtggcaatccggtcagcgtggaggttcagtccgtcaccgacggcgtgaaggtaaaagtgagccgtgttcctgacggtgttgctgaatacagcgtatgggagctgaagctgccgacgctgcgccagcgactgttccgctgcgtgagtatccgtgagaacgacgacggcacgtatgccatcaccgccgtgcagcatgtgccggaaaaagaggccatcgtggataacggggcgcactttgacggcgaacagagtggcacggtgaatggtgtcacgccgccagcggtgcagcacctgaccgcagaagtcactgcagacagcggggaatatcaggtgctggcgcgatgggacacaccgaaggtggtgaagggcgtgagtttcctgctccgtctgaccgtaacagcggacgacggcagtgagcggctggtcagcacggcccggacgacggaaaccacataccgcttcacgcaactggcgctggggaactacaggctgacagtccgggcggtaaatgcgtgggggcagcagggcgatccggcgtcggtatcgttccggattgccgcaccggcagcaccgtcgaggattgagctgacgccgggctattttcagataaccgccacgccgcatcttgccgtttatgacccgacggtacagtttgagttctggttctcggaaaagcagattgcggatatcagacaggttgaaaccagcacgcgttatcttggtacggcgctgtactggatagccgccagtatcaatatcaaaccgggccatgattattacttttatatccgcagtgtgaacaccgttggcaaatcggcattcgtggaggccgtcggtcgggcgagcgatgatgcggaaggttacctggattttttcaaaggcaagataaccgaatcccatctcggcaaggagctgctggaaaaagtcgagctgacggaggataacgccagcagactggaggagttttcgaaagagtggaaggatgccagtgataagtggaatgccatgtgggctgtcaaaattgagcagaccaaagacggcaaacattatgtcgcgggtattggcctcagcatggaggacacggaggaaggcaaactgagccagtttctggttgccgccaatcgtatcgcatttattgacccggcaaacgggaatgaaacgccgatgtttgtggcgcagggcaaccagatattcatgaacgacgtgttcctgaagcgcctgacggcccccaccattaccagcggcggcaatcctccggccttttccctgacaccggacggaaagctgaccgctaaaaatgcggatatcagtggcagtgtgaatgcgaactccgggacgctcagtaatgtgacgatagctgaaaactgtacgataaacggtacgctgagggcggaaaaaatcgtcggggacattgtaaaggcggcgagcgcggcttttccgcgccagcgtgaaagcagtgtggactggccgtcaggtacccgtactgtcaccgtgaccgatgaccatccttttgatcgccagatagtggtgcttccgctgacgtttcgcggaagtaagcgtactgtcagcggcaggacaacgtattcgatgtgttatctgaaagtactgatgaacggtgcggtgatttatgatggcgcggcgaacgaggcggtacaggtgttctcccgtattgttgacatgccagcgggtcggggaaacgtgatcctgacgttcacgcttacgtccacacggcattcggcagatattccgccgtatacgtttgccagcgatgtgcaggttatggtgattaagaaacaggcgctgggcatcagcgtggtctgagtgtgttacagaggttcgtccgggaacgggcgttttattataaaacagtgagaggtgaacgatgcgtaatgtgtgtattgccgttgctgtctttgccgcacttgcggtgacagtcactccggcccgtgcggaaggtggacatggtacgtttacggtgggctattttcaagtgaaaccgggtacattgccgtcgttgtcgggcggggataccggtgtgagtcatctgaaagggattaacgtgaagtaccgttatgagctgacggacagtgtgggggtgatggcttccctggggttcgccgcgtcgaaaaagagcagcacagtgatgaccggggaggatacgtttcactatgagagcctgcgtggacgttatgtgagcgtgatggccggaccggttttacaaatcagtaagcaggtcagtgcgtacgccatggccggagtggctcacagtcggtggtccggcagtacaatggattaccgtaagacggaaatcactcccgggtatatgaaagagacgaccactgccagggacgaaagtgcaatgcggcatacctcagtggcgtggagtgcaggtatacagattaatccggcagcgtccgtcgttgttgatattgcttatgaaggctccggcagtggcgactggcgtactgacggattcatcgttggggtcggttataaattctgattagccaggtaacacagtgttatgacagcccgccggaaccggtgggcttttttgtggggtgaatatggcagtaaagatttcaggagtcctgaaagacggcacaggaaaaccggtacagaactgcaccattcagctgaaagccagacgtaacagcaccacggtggtggtgaacacggtgggctcagagaatccggatgaagccgggcgttacagcatggatgtggagtacggtcagtacagtgtcatcctgcaggttgacggttttccaccatcgcacgccgggaccatcaccgtgtatgaagattcacaaccggggacgctgaatgattttctctgtgccatgacggaggatgatgcccggccggaggtgctgcgtcgtcttgaactgatggtggaagaggtggcgcgtaacgcgtccgtggtggcacagagtacggcagacgcgaagaaatcagccggcgatgccagtgcatcagctgctcaggtcgcggcccttgtgactgatgcaactgactcagcacgcgccgccagcacgtccgccggacaggctgcatcgtcagctcaggaagcgtcctccggcgcagaagcggcatcagcaaaggccactgaagcggaaaaaagtgccgcagccgcagagtcctcaaaaaacgcggcggccaccagtgccggtgcggcgaaaacgtcagaaacgaatgctgcagcgtcacaacaatcagccgccacgtctgcctccaccgcggccacgaaagcgtcagaggccgccacttcagcacgagatgcggtggcctcaaaagaggcagcaaaatcatcagaaacgaacgcatcatcaagtgccggtcgtgcagcttcctcggcaacggcggcagaaaattctgccagggcggcaaaaacgtccgagacgaatgccaggtcatctgaaacagcagcggaacggagcgcctctgccgcggcagacgcaaaaacagcggcggcggggagtgcgtcaacggcatccacgaaggcgacagaggctgcgggaagtgcggtatcagcatcgcagagcaaaagtgcggcagaagcggcggcaatacgtgcaaaaaattcggcaaaacgtgcagaagatatagcttcagctgtcgcgcttgaggatgcggacacaacgagaaaggggatagtgcagctcagcagtgcaaccaacagcacgtctgaaacgcttgctgcaacgccaaaggcggttaaggtggtaatggatgaaacgaacagaaaagcccactggacagtccggcactgaccggaacgccaacagcaccaaccgcgctcaggggaacaaacaatacccagattgcgaacaccgcttttgtactggccgcgattgcagatgttatcgacgcgtcacctgacgcactgaatacgctgaatgaactggccgcagcgctcgggaatgatccagattttgctaccaccatgactaacgcgcttgcgggtaaacaaccgaagaatgcgacactgacggcgctggcagggctttccacggcgaaaaataaattaccgtattttgcggaaaatgatgccgccagcctgactgaactgactcaggttggcagggatattctggcaaaaaattccgttgcagatgttcttgaataccttggggccggtgagaattcggcctttccggcaggtgcgccgatcccgtggccatcagatatcgttccgtctggctacgtcctgatgcaggggcaggcgtttgacaaatcagcctacccaaaacttgctgtcgcgtatccatcgggtgtgcttcctgatatgcgaggctggacaatcaaggggaaacccgccagcggtcgtgctgtattgtctcaggaacaggatggaattaagtcgcacacccacagtgccagtgcatccggtacggatttggggacgaaaaccacatcgtcgtttgattacgggacgaaaacaacaggcagtttcgattacggcaccaaatcgacgaataacacgggggctcatgctcacagtctgagcggttcaacaggggccgcgggtgctcatgcccacacaagtggtttaaggatgaacagttctggctggagtcagtatggaacagcaaccattacaggaagtttatccacagttaaaggaaccagcacacagggtattgcttatttatcgaaaacggacagtcagggcagccacagtcactcattgtccggtacagccgtgagtgccggtgcacatgcgcatacagttggtattggtgcgcaccagcatccggttgttatcggtgctcatgcccattctttcagtattggttcacacggacacaccatcaccgttaacgctgcgggtaacgcggaaaacaccgtcaaaaacattgcatttaactatattgtgaggcttgcataatggcattcagaatgagtgaacaaccacggaccataaaaatttataatctgctggccggaactaatgaatttattggtgaaggtgacgcatatattccgcctcataccggtctgcctgcaaacagtaccgatattgcaccgccagatattccggctggctttgtggctgttttcaacagtgatgaggcatcgtggcatctcgttgaagaccatcggggtaaaaccgtctatgacgtggcttccggcgacgcgttatttatttctgaactcggtccgttaccggaaaattttacctggttatcgccgggaggggaatatcagaagtggaacggcacagcctgggtgaaggatacggaagcagaaaaactgttccggatccgggaggcggaagaaacaaaaaaaagcctgatgcaggtagccagtgagcatattgcgccgcttcaggatgctgcagatctggaaattgcaacgaaggaagaaacctcgttgctggaagcctggaagaagtatcgggtgttgctgaaccgtgttgatacatcaactgcacctgatattgagtggcctgctgtccctgttatggagtaatcgttttgtgatatgccgcagaaacgttgtatgaaataacgttctgcggttagttagtatattgtaaagctgagtattggtttatttggcgattattatcttcaggagaataatggaagttctatgactcaattgttcatagtgtttacatcaccgccaattgcttttaagactgaacgcatgaaatatggtttttcgtcatgttttgagtctgctgttgatatttctaaagtcggttttttttcttcgttttctctaactattttccatgaaatacatttttgattattatttgaatcaattccaattacctgaagtctttcatctataattggcattgtatgtattggtttattggagtagatgcttgcttttctgagccatagctctgatatccaaatgaagccataggcatttgttattttggctctgtcagctgcataacgccaaaaaatatatttatctgcttgatcttcaaatgttgtattgattaaatcaattggatggaattgtttatcataaaaaattaatgtttgaatgtgataaccgtcctttaaaaaagtcgtttctgcaagcttggctgtatagtcaactaactcttctgtcgaagtgatatttttaggcttatctaccagttttagacgctctttaatatcttcaggaattattttattgtcatattgtatcatgctaaatgacaatttgcttatggagtaatcttttaattttaaataagttattctcctggcttcatcaaataaagagtcgaatgatgttggcgaaatcacatcgtcacccattggattgtttatttgtatgccaagagagttacagcagttatacattctgccatagattatagctaaggcatgtaataattcgtaatcttttagcgtattagcgacccatcgtctttctgatttaataatagatgattcagttaaatatgaaggtaatttcttttgtgcaagtctgactaacttttttataccaatgtttaacatactttcatttgtaataaactcaatgtcattttcttcaatgtaagatgaaataagagtagcctttgcctcgctatacatttctaaatcgccttgtttttctatcgtattgcgagaatttttagcccaagccattaatggatcatttttccatttttcaataacattattgttataccaaatgtcatatcctataatctggtttttgtttttttgaataataaatgttactgttcttgcggtttggaggaattgattcaaattcaagcgaaataattcagggtcaaaatatgtatcaatgcagcatttgagcaagtgcgataaatctttaagtcttctttcccatggttttttagtcataaaactctccattttgataggttgcatgctagatgctgatatattttagaggtgataaaattaactgcttaactgtcaatgtaatacaagttgtttgatctttgcaatgattcttatcagaaaccatatagtaaattagttacacaggaaatttttaatattattattatcattcattatgtattaaaattagagttgtggcttggctctgctaacacgttgctcataggagatatggtagagccgcagacacgtcgtatgcaggaacgtgctgcggctggctggtgaacttccgatagtgcgggtgttgaatgatttccagttgctaccgattttacatattttttgcatgagagaatttgtaccacctcccaccgaccatctatgactgtacgccactgtccctaggactgctatgtgccggagcggacattacaaacgtccttctcggtgcatgccactgttgccaatgacctgcctaggaattggttagcaagttactaccggattttgtaaaaacagccctcctcatataaaaagtattcgttcacttccgataagcgtcgtaattttctatctttcatcatattctagatccctctgaaaaaatcttccgagtttgctaggcactgatacataactcttttccaataattggggaagtcattcaaatctataataggtttcagatttgcttcaataaattctgactgtagctgctgaaacgttgcggttgaactatatttccttataacttttacgaaagagtttctttgagtaatcacttcactcaagtgcttccctgcctccaaacgatacctgttagcaatatttaatagcttgaaatgatgaagagctctgtgtttgtcttcctgcctccagttcgccgggcattcaacataaaaactgatagcacccggagttccggaaacgaaatttgcatatacccattgctcacgaaaaaaaatgtccttgtcgatatagggatgaatcgcttggtgtacctcatctactgcgaaaacttgacctttctctcccatattgcagtcgcggcacgatggaactaaattaataggcatcaccgaaaattcaggataatgtgcaataggaagaaaatgatctatattttttgtctgtcctatatcaccacaaaatggacatttttcacctgatgaaacaagcatgtcatcgtaatatgttctagcgggtttgtttttatctcggagattattttcataaagcttttctaatttaacctttgtcaggttaccaactactaaggttgtaggctcaagagggtgtgtcctgtcgtaggtaaataactgacctgtcgagcttaatattctatattgttgttctttctgcaaaaaagtggggaagtgagtaatgaaattatttctaacatttatctgcatcataccttccgagcatttattaagcatttcgctataagttctcgctggaagaggtagttttttcattgtactttaccttcatctctgttcattatcatcgcttttaaaacggttcgaccttctaatcctatctgaccattataattttttagaatggtttcataagaaagctctgaatcaacggactgcgataataagtggtggtatccagaatttgtcacttcaagtaaaaacacctcacgagttaaaacacctaagttctcaccgaatgtctcaatatccggacggataatatttattgcttctcttgaccgtaggactttccacatgcaggattttggaacctcttgcagtactactggggaatgagttgcaattattgctacaccattgcgtgcatcgagtaagtcgcttaatgttcgtaaaaaagcagagagcaaaggtggatgcagatgaacctctggttcatcgaataaaactaatgacttttcgccaacgacatctactaatcttgtgatagtaaataaaacaattgcatgtccagagctcattcgaagcagatatttctggatattgtcataaaacaatttagtgaatttatcatcgtccacttgaatctgtggttcattacgtcttaactcttcatatttagaaatgaggctgatgagttccatatttgaaaagttttcatcactacttagttttttgatagcttcaagccagagttgtctttttctatctactctcatacaaccaataaatgctgaaatgaattctaagcggagatcgcctagtgattttaaactattgctggcagcattcttgagtccaatataaaagtattgtgtaccttttgctgggtcaggttgttctttaggaggagtaaaaggatcaaatgcactaaacgaaactgaaacaagcgatcgaaaatatccctttgggattcttgactcgataagtctattattttcagagaaaaaatattcattgttttctgggttggtgattgcaccaatcattccattcaaaattgttgttttaccacacccattccgcccgataaaagcatgaatgttcgtgctgggcatagaattaaccgtcacctcaaaaggtatagttaaatcactgaatccgggagcactttttctattaaatgaaaagtggaaatctgacaattctggcaaaccatttaacacacgtgcgaactgtccatgaatttctgaaagagttacccctctaagtaatgaggtgttaaggacgctttcattttcaatgtcggctaatcgatttggccatactactaaatcctgaatagctttaagaaggttatgtttaaaaccatcgcttaatttgctgagattaacatagtagtcaatgctttcacctaaggaaaaaaacatttcagggagttgactgaattttttatctattaatgaataagtgcttacttcttctttttgacctacaaaaccaattttaacatttccgatatcgcatttttcaccatgctcatcaaagacagtaagataaaacattgtaacaaaggaatagtcattccaaccatctgctcgtaggaatgccttatttttttctactgcaggaatatacccgcctctttcaataacactaaactccaacatatagtaacccttaattttattaaaataaccgcaatttatttggcggcaacacaggatctctcttttaagttactctctattacatacgttttccatctaaaaattagtagtattgaacttaacggggcatcgtattgtagttttccatatttagctttctgcttccttttggataacccactgttattcatgttgcatggtgcactgtttataccaacgatatagtctattaatgcatatatagtatcgccgaacgattagctcttcaggcttctgaagaagcgtttcaagtactaataagccgatagatagccacggacttcgtagccatttttcataagtgttaacttccgctcctcgctcataacagacattcactacagttatggcggaaaggtatgcatgctgggtgtggggaagtcgtgaaagaaaagaagtcagctgcgtcgtttgacatcactgctatcttcttactggttatgcaggtcgtagtgggtggcacacaaagctttgcactggattgcgaggctttgtgcttctctggagtgcgacaggtttgatgacaaaaaattagcgcaagaagacaaaaatcaccttgcgctaatgctctgttacaggtcactaataccatctaagtagttgattcatagtgactgcatatgttgtgttttacagtattatgtagtctgttttttatgcaaaatctaatttaatatattgatatttatatcattttacgtttctcgttcagcttttttatactaagttggcattataaaaaagcattgcttatcaatttgttgcaacgaacaggtcactatcagtcaaaataaaatcattatttgatttcaattttgtcccactccctgcctctgtcatcacgatactgtgatgccatggtgtccgacttatgcccgagaagatgttgagcaaacttatcgcttatctgcttctcatagagtcttgcagacaaactgcgcaactcgtgaaaggtaggcggatccccttcgaaggaaagacctgatgcttttcgtgcgcgcataaaataccttgatactgtgccggatgaaagcggttcgcgacgagtagatgcaattatggtttctccgccaagaatctctttgcatttatcaagtgtttccttcattgatattccgagagcatcaatatgcaatgctgttgggatggcaatttttacgcctgttttgctttgctcgacataaagatatccatctacgatatcagaccacttcatttcgcataaatcaccaactcgttgcccggtaacaacagccagttccattgcaagtctgagccaacatggtgatgattctgctgcttgataaattttcaggtattcgtcagccgtaagtcttgatctccttacctctgattttgctgcgcgagtggcagcgacatggtttgttgttatatggccttcagctattgcctctcggaatgcatcgctcagtgttgatctgattaacttggctgacgccgccttgccctcgtctatgtatccattgagcattgccgcaatttcttttgtggtgatgtcttcaagtggagcatcaggcagacccctccttattgctttaattttgctcatgtaatttatgagtgtcttctgcttgattcctctgctggccaggattttttcgtagcgatcaagccatgaatgtaacgtaacggaattatcactgttgattctcgctgtcagaggcttgtgtttgtgtcctgaaaataactcaatgttggcctgtatagcttcagtgattgcgattcgcctgtctctgcctaatccaaactctttacccgtccttgggtccctgtagcagtaatatccattgtttcttatataaaggttagggggtaaatcccggcgctcatgacttcgccttcttcccatttctgatcctcttcaaaaggccacctgttactggtcgatttaagtcaacctttaccgctgattcgtggaacagatactctcttccatccttaaccggaggtgggaatatcctgcattcccgaacccatcgacgaactgtttcaaggcttcttggacgtcgctggcgtgcgttccactcctgaagtgtcaagtacatcgcaaagtctccgcaattacacgcaagaaaaaaccgccatcaggcggcttggtgttctttcagttcttcaattcgaatattggttacgtctgcatgtgctatctgcgcccatatcatccagtggtcgtagcagtcgttgatgttctccgcttcgataactctgttgaatggctctccattccattctcctgtgactcggaagtgcatttatcatctccataaaacaaaacccgccgtagcgagttcagataaaataaatccccgcgagtgcgaggattgttatgtaatattgggtttaatcatctatatgttttgtacagagagggcaagtatcgtttccaccgtactcgtgataataattttgcacggtatcagtcatttctcgcacattgcagaatggggatttgtcttcattagacttataaaccttcatggaatatttgtatgccgactctatatctataccttcatctacataaacaccttcgtgatgtctgcatggagacaagacaccggatctgcacaacattgataacgcccaatctttttgctcagactctaactcattgatactcatttataaactccttgcaatgtatgtcgtttcagctaaacggtatcagcaatgtttatgtaaagaaacagtaagataatactcaacccgatgtttgagtacggtcatcatctgacactacagactctggcatcgctgtgaagacgacgcgaaattcagcattttcacaagcgttatcttttacaaaaccgatctcactctcctttgatgcgaatgccagcgtcagacatcatatgcagatactcacctgcatcctgaacccattgacctccaaccccgtaatagcgatgcgtaatgatgtcgatagttactaacgggtcttgttcgattaactgccgcagaaactcttccaggtcaccagtgcagtgcttgataacaggagtcttcccaggatggcgaacaacaagaaactggtttccgtcttcacggacttcgttgctttccagtttagcaatacgcttactcccatccgagataacaccttcgtaatactcacgctgctcgttgagttttgattttgctgtttcaagctcaacacgcagtttccctactgttagcgcaatatcctcgttctcctggtcgcggcgtttgatgtattgctggtttctttcccgttcatccagcagttccagcacaatcgatggtgttaccaattcatggaaaaggtctgcgtcaaatccccagtcgtcatgcattgcctgctctgccgcttcacgcagtgcctgagagttaatttcgctcacttcgaacctctctgtttactgataagttccagatcctcctggcaacttgcacaagtccgacaaccctgaacgaccaggcgtcttcgttcatctatcggatcgccacactcacaacaatgagtggcagatatagcctggtggttcaggcggcgcatttttattgctgtgttgcgctgtaattcttctatttctgatgctgaatcaatgatgtctgccatctttcattaatccctgaactgttggttaatacgcttgagggtgaatgcgaataataaaaaaggagcctgtagctccctgatgattttgcttttcatgttcatcgttccttaaagacgccgtttaacatgccgattgccaggcttaaatgagtcggtgtgaatcccatcagcgttaccgtttcgcggtgcttcttcagtacgctacggcaaatgtcatcgacgtttttatccggaaactgctgtctggctttttttgatttcagaattagcctgacgggcaatgctgcgaagggcgttttcctgctgaggtgtcattgaacaagtcccatgtcggcaagcataagcacacagaatatgaagcccgctgccagaaaaatgcattccgtggttgtcatacctggtttctctcatctgcttctgctttcgccaccatcatttccagcttttgtgaaagggatgcggctaacgtatgaaattcttcgtctgtttctactggtattggcacaaacctgattccaatttgagcaaggctatgtgccatctcgatactcgttcttaactcaacagaagatgctttgtgcatacagcccctcgtttattatttatctcctcagccagccgctgtgctttcagtggatttcggataacagaaaggccgggaaatacccagcctcgctttgtaacggagtagacgaaagtgattgcgcctacccggatattatcgtgaggatgcgtcatcgccattgctccccaaatacaaaaccaatttcagccagtgcctcgtccattttttcgatgaactccggcacgatctcgtcaaaactcgccatgtacttttcatcccgctcaatcacgacataatgcaggccttcacgcttcatacgcgggtcatagttggcaaagtaccaggcattttttcgcgtcacccacatgctgtactgcacctgggccatgtaagctgactttatggcctcgaaaccaccgagccggaacttcatgaaatcccgggaggtaaacgggcatttcagttcaaggccgttgccgtcactgcataaaccatcgggagagcaggcggtacgcatactttcgtcgcgatagatgatcggggattcagtaacattcacgccggaagtgaattcaaacagggttctggcgtcgttctcgtactgttttccccaggccagtgctttagcgttaacttccggagccacaccggtgcaaacctcagcaagcagggtgtggaagtaggacattttcatgtcaggccacttctttccggagcggggttttgctatcacgttgtgaacttctgaagcggtgatgacgccgagccgtaatttgtgccacgcatcatccccctgttcgacagctctcacatcgatcccggtacgctgcaggataatgtccggtgtcatgctgccaccttctgctctgcggctttctgtttcaggaatccaagagcttttactgcttcggcctgtgtcagttctgacgatgcacgaatgtcgcggcgaaatatctgggaacagagcggcaataagtcgtcatcccatgttttatccagggcgatcagcagagtgttaatctcctgcatggtttcatcgttaaccggagtgatgtcgcgttccggctgacgttctgcagtgtatgcagtattttcgacaatgcgctcggcttcatccttgtcatagataccagcaaatccgaaggccagacgggcacactgaatcatggctttatgacgtaacatccgtttgggatgcgactgccacggccccgtgatttctctgccttcgcgagttttgaatggttcgcggcggcattcatccatccattcggtaacgcagatcggatgattacggtccttgcggtaaatccggcatgtacaggattcattgtcctgctcaaagtccatgccatcaaactgctggttttcattgatgatgcgggaccagccatcaacgcccaccaccggaacgatgccattctgcttatcaggaaaggcgtaaatttctttcgtccacggattaaggccgtactggttggcaacgatcagtaatgcgatgaactgcgcatcgctggcatcacctttaaatgccgtctggcgaagagtggtgatcagttcctgtgggtcgacagaatccatgccgacacgttcagccagcttcccagccagcgttgcgagtgcagtactcattcgttttatacctctgaatcaatatcaacctggtggtgagcaatggtttcaaccatgtaccggatgtgttctgccatgcgctcctgaaactcaacatcgtcatcaaacgcacgggtaatggattttttgctggccccgtggcgttgcaaatgatcgatgcatagcgattcaaacaggtgctggggcaggcctttttccatgtcgtctgccagttctgcctctttctcttcacgggcgagctgctggtagtgacgcgcccagctctgagcctcaagacgatcctgaatgtaataagcgttcatggctgaactcctgaaatagctgtgaaaatatcgcccgcgaaatgccgggctgattaggaaaacaggaaagggggttagtgaatgcttttgcttgatctcagtttcagtattaatatccattttttataagcgtcgacggcttcacgaaacatcttttcatcgccaataaaagtggcgatagtgaatttagtctggatagccataagtgtttgatccattctttgggactcctggctgattaagtatgtcgataaggcgtttccatccgtcacgtaatttacgggtgattcgttcaagtaaagattcggaagggcagccagcaacaggccaccctgcaatggcatattgcatggtgtgctccttatttatacataacgaaaaacgcctcgagtgaagcgttattggtatgcggtaaaaccgcactcaggcggccttgatagtcatatcatctgaatcaaatattcctgatgtatcgatatcggtaattcttattccttcgctaccatccattggaggccatccttcctgaccatttccatcattccagtcgaactcacacacaacaccatatgcatttaagtcgcttgaaattgctataagcagagcatgttgcgccagcatgattaatacagcatttaatacagagccgtgtttattgagtcggtattcagagtctgaccagaaattattaatctggtgaagtttttcctctgtcattacgtcatggtcgatttcaatttctattgatgctttccagtcgtaatcaatgatgtattttttgatgtttgacatctgttcatatcctcacagataaaaaatcgccctcacactggagggcaaagaagatttccaataatcagaacaagtcggctcctgtttagttacgagcgacattgctccgtgtattcactcgttggaatgaatacacagtgcagtgtttattctgttatttatgccaaaaataaaggccactatcaggcagctttgttgttctgtttaccaagttctctggcaatcattgccgtcgttcgtattgcccatttatcgacatatttcccatcttccattacaggaaacatttcttcaggcttaaccatgcattccgattgcagcttgcatccattgcatcgcttgaattgtccacaccattgatttttatcaatagtcgtagtcatacggatagtcctggtattgttccatcacatcctgaggatgctcttcgaactcttcaaattcttcttccatatatcaccttaaatagtggattgcggtagtaaagattgtgcctgtcttttaaccacatcaggctcggtggttctcgtgtacccctacagcgagaaatcggataaactattacaacccctacagtttgatgagtatagaaatggatccactcgttattctcggacgagtgttcagtaatgaacctctggagagaaccatgtatatgatcgttatctgggttggacttctgcttttaagcccagataactggcctgaatatgttaatgagagaatcggtattcctcatgtgtggcatgttttcgtctttgctcttgcattttcgctagcaattaatgtgcatcgattatcagctattgccagcgccagatataagcgatttaagctaagaaaacgcattaagatgcaaaacgataaagtgcgatcagtaattcaaaaccttacagaagagcaatctatggttttgtgcgcagcccttaatgaaggcaggaagtatgtggttacatcaaaacaattcccatacattagtgagttgattgagcttggtgtgttgaacaaaactttttcccgatggaatggaaagcatatattattccctattgaggatatttactggactgaattagttgccagctatgatccatataatattgagataaagccaaggccaatatctaagtaactagataagaggaatcgattttcccttaattttctggcgtccactgcatgttatgccgcgttcgccaggcttgctgtaccatgtgcgctgattcttgcgctcaatacgttgcaggttgctttcaatctgtttgtggtattcagccagcactgtaaggtctatcggatttagtgcgctttctactcgtgatttcggtttgcgattcagcgagagaatagggcggttaactggttttgcgcttaccccaaccaacaggggatttgctgctttccattgagcctgtttctctgcgcgacgttcgcggcggcgtgtttgtgcatccatctggattctcctgtcagttagctttggtggtgtgtggcagttgtagtcctgaacgaaaaccccccgcgattggcacattggcagctaatccggaatcgcacttacggccaatgcttcgtttcgtatcacacaccccaaagccttctgctttgaatgctgcccttcttcagggcttaatttttaagagcgtcaccttcatggtggtcagtgcgtcctgctgatgtgctcagtatcaccgccagtggtatttatgtcaacaccgccagagataatttatcaccgcagatggttatctgtatgttttttatatgaatttattttttgcaggggggcattgtttggtaggtgagagatctgaattgctatgtttagtgagttgtatctatttatttttcaataaatacaattggttatgtgttttgggggcgatcgtgaggcaaagaaaacccggcgctgaggccgggttattcttgttctctggtcaaattatatagttggaaaacaaggatgcatatatgaatgaacgatgcagaggcaatgccgatggcgatagtgggtatcatgtagccgcttatgctggaaagaagcaataacccgcagaaaaacaaagctccaagctcaacaaaactaagggcatagacaataactaccgatgtcatatacccatactctctaatcttggccagtcggcgcgttctgcttccgattagaaacgtcaaggcagcaatcaggattgcaatcatggttcctgcatatgatgacaatgtcgccccaagaccatctctatgagctgaaaaagaaacaccaggaatgtagtggcggaaaaggagatagcaaatgcttacgataacgtaaggaattattactatgtaaacaccaggcatgattctgttccgcataattactcctgataattaatccttaactttgcccacctgccttttaaaacattccagtatatcacttttcattcttgcgtagcaatatgccatctcttcagctatctcagcattggtgaccttgttcagaggcgctgagagatggcctttttctgatagataatgttctgttaaaatatctccggcctcatcttttgcccgcaggctaatgtctgaaaattgaggtgacgggttaaaaataatatccttggcaaccttttttatatcccttttaaattttggcttaatgactatatccaatgagtcaaaaagctccccttcaatatctgttgcccctaagacctttaatatatcgccaaatacaggtagcttggcttctaccttcaccgttgttcggccgatgaaatgcatatgcataacatcgtctttggtggttcccctcatcagtggctctatctgaacgcgctctccactgcttaatgacattcctttcccgattaaaaaatctgtcagatcggatgtggtcggcccgaaaacagttctggcaaaaccaatggtgtcgccttcaacaaacaaaaaagatgggaatcccaatgattcgtcatctgcgaggctgttcttaatatcttcaactgaagctttagagcgatttatcttctgaaccagactcttgtcatttgttttggtaaagagaaaagtttttccatcgattttatgaatatacaaataattggagccaacctgcaggtgatgattatcagccagcagagaattaaggaaaacagacaggtttattgagcgcttatctttccctttatttttgctgcggtaagtcgcataaaaaccattcttcataattcaatccatttactatgttatgttctgaggggagtgaaaattcccctaattcgatgaagattcttgctcaattgttatcagctatgcgccgaccagaacaccttgccgatcagccaaacgtctcttcaggccactgactagcgataactttccccacaacggaacaactctcattgcatgggatcattgggtactgtgggtttagtggttgtaaaaacacctgaccgctatccctgatcagtttcttgaaggtaaactcatcacccccaagtctggctatgcagaaatcacctggctcaacagcctgctcagggtcaacgagaattaacattccgtcaggaaagcttggcttggagcctgttggtgcggtcatggaattaccttcaacctcaagccagaatgcagaatcactggcttttttggttgtgcttacccatctctccgcatcacctttggtaaaggttctaagctcaggtgagaacatccctgcctgaacatgagaaaaaacagggtactcatactcacttctaagtgacggctgcatactaaccgcttcatacatctcgtagatttctctggcgattgaagggctaaattcttcaacgctaactttgagaatttttgcaagcaatgcggcgttataagcatttaatgcattgatgccattaaataaagcaccaacgcctgactgccccatccccatcttgtctgcgacagattcctgggataagccaagttcatttttctttttttcataaattgctttaaggcgacgtgcgtcctcaagctgctcttgtgttaatggtttcttttttgtgctcatacgttaaatctatcaccgcaagggataaatatctaacaccgtgcgtgttgactattttacctctggcggtgataatggttgcatgtactaaggaggttgtatggaacaacgcataaccctgaaagattatgcaatgcgctttgggcaaaccaagacagctaaagatctcggcgtatatcaaagcgcgatcaacaaggccattcatgcaggccgaaagatttttttaactataaacgctgatggaagcgtttatgcggaagaggtaaagcccttcccgagtaacaaaaaaacaacagcataaataaccccgctcttacacattccagccctgaaaaagggcatcaaattaaaccacacctatggtgtatgcatttatttgcatacattcaatcaattgttatctaaggaaatacttacatatggttcgtgcaaacaaacgcaacgaggctctacgaatcgagagtgcgttgcttaacaaaatcgcaatgcttggaactgagaagacagcggaagctgtgggcgttgataagtcgcagatcagcaggtggaagagggactggattccaaagttctcaatgctgcttgctgttcttgaatggggggtcgttgacgacgacatggctcgattggcgcgacaagttgctgcgattctcaccaataaaaaacgcccggcggcaaccgagcgttctgaacaaatccagatggagttctgaggtcattactggatctatcaacaggagtcattatgacaaatacagcaaaaatactcaacttcggcagaggtaactttgccggacaggagcgtaatgtggcagatctcgatgatggttacgccagactatcaaatatgctgcttgaggcttattcgggcgcagatctgaccaagcgacagtttaaagtgctgcttgccattctgcgtaaaacctatgggtggaataaaccaatggacagaatcaccgattctcaacttagcgagattacaaagttacctgtcaaacggtgcaatgaagccaagttagaactcgtcagaatgaatattatcaagcagcaaggcggcatgtttggaccaaataaaaacatctcagaatggtgcatccctcaaaacgagggaaaatcccctaaaacgagggataaaacatccctcaaattgggggattgctatccctcaaaacagggggacacaaaagacactattacaaaagaaaaaagaaaagattattcgtcagagaattctggcgaatcctctgaccagccagaaaacgacctttctgtggtgaaaccggatgctgcaattcagagcggcagcaagtgggggacagcagaagacctgaccgccgcagagtggatgtttgacatggtgaagactatcgcaccatcagccagaaaaccgaattttgctgggtgggctaacgatatccgcctgatgcgtgaacgtgacggacgtaaccaccgcgacatgtgtgtgctgttccgctgggcatgccaggacaacttctggtccggtaacgtgctgagcccggccaaactccgcgataagtggacccaactcgaaatcaaccgtaacaagcaacaggcaggcgtgacagccagcaaaccaaaactcgacctgacaaacacagactggatttacggggtggatctatgaaaaacatcgccgcacagatggttaactttgaccgtgagcagatgcgtcggatcgccaacaacatgccggaacagtacgacgaaaagccgcaggtacagcaggtagcgcagatcatcaacggtgtgttcagccagttactggcaactttcccggcgagcctggctaaccgtgaccagaacgaagtgaacgaaatccgtcgccagtgggttctggcttttcgggaaaacgggatcaccacgatggaacaggttaacgcaggaatgcgcgtagcccgtcggcagaatcgaccatttctgccatcacccgggcagtttgttgcatggtgccgggaagaagcatccgttaccgccggactgccaaacgtcagcgagctggttgatatggtttacgagtattgccggaagcgaggcctgtatccggatgcggagtcttatccgtggaaatcaaacgcgcactactggctggttaccaacctgtatcagaacatgcgggccaatgcgcttactgatgcggaattacgccgtaaggccgcagatgagcttgtccatatgactgcgagaattaaccgtggtgaggcgatccctgaaccagtaaaacaacttcctgtcatgggcggtagacctctaaatcgtgcacaggctctggcgaagatcgcagaaatcaaagctaagttcggactgaaaggagcaagtgtatgacgggcaaagaggcaattattcattacctggggacgcataatagcttctgtgcgccggacgttgccgcgctaacaggcgcaacagtaaccagcataaatcaggccgcggctaaaatggcacgggcaggtcttctggttatcgaaggtaaggtctggcgaacggtgtattaccggtttgctaccagggaagaacgggaaggaaagatgagcacgaacctggtttttaaggagtgtcgccagagtgccgcgatgaaacgggtattggcggtatatggagttaaaagatgaccatctacattactgagctaataacaggcctgctggtaatcgcaggcctttttatttgggggagagggaagtcatgaaaaaactaacctttgaaattcgatctccagcacatcagcaaaacgctattcacgcagtacagcaaatccttccagacccaaccaaaccaatcgtagtaaccattcaggaacgcaaccgcagcttagaccaaaacaggaagctatgggcctgcttaggtgacgtctctcgtcaggttgaatggcatggtcgctggctggatgcagaaagctggaagtgtgtgtttaccgcagcattaaagcagcaggatgttgttcctaaccttgccgggaatggctttgtggtaataggccagtcaaccagcaggatgcgtgtaggcgaatttgcggagctattagagcttatacaggcattcggtacagagcgtggcgttaagtggtcagacgaagcgagactggctctggagtggaaagcgagatggggagacagggctgcatgataaatgtcgttagtttctccggtggcaggacgtcagcatatttgctctggctaatggagcaaaagcgacgggcaggtaaagacgtgcattacgttttcatggatacaggttgtgaacatccaatgacatatcggtttgtcagggaagttgtgaagttctgggatataccgctcaccgtattgcaggttgatatcaacccggagcttggacagccaaatggttatacggtatgggaaccaaaggatattcagacgcgaatgcctgttctgaagccatttatcgatatggtaaagaaatatggcactccatacgtcggcggcgcgttctgcactgacagattaaaactcgttcccttcaccaaatactgtgatgaccatttcgggcgagggaattacaccacgtggattggcatcagagctgatgaaccgaagcggctaaagccaaagcctggaatcagatatcttgctgaactgtcagactttgagaaggaagatatcctcgcatggtggaagcaacaaccattcgatttgcaaataccggaacatctcggtaactgcatattctgcattaaaaaatcaacgcaaaaaatcggacttgcctgcaaagatgaggagggattgcagcgtgtttttaatgaggtcatcacgggatcccatgtgcgtgacggacatcgggaaacgccaaaggagattatgtaccgaggaagaatgtcgctggacggtatcgcgaaaatgtattcagaaaatgattatcaagccctgtatcaggacatggtacgagctaaaagattcgataccggctcttgttctgagtcatgcgaaatatttggagggcagcttgatttcgacttcgggagggaagctgcatgatgcgatgttatcggtgcggtgaatgcaaagaagataaccgcttccgaccaaatcaaccttactggaatcgatggtgtctccggtgtgaaagaacaccaacaggggtgttaccactaccgcaggaaaaggaggacgtgtggcgagacagcgacgaagtatcaccgacataatctgcgaaaactgcaaataccttccaacgaaacgcaccagaaataaacccaagccaatcccaaaagaatctgacgtaaaaaccttcaactacacggctcacctgtgggatatccggtggctaagacgtcgtgcgaggaaaacaaggtgattgaccaaaatcgaagttacgaacaagaaagcgtcgagcgagctttaacgtgcgctaactgcggtcagaagctgcatgtgctggaagttcacgtgtgtgagcactgctgcgcagaactgatgagcgatccgaatagctcgatgcacgaggaagaagatgatggctaaaccagcgcgaagacgatgtaaaaacgatgaatgccgggaatggtttcaccctgcattcgctaatcagtggtggtgctctccagagtgtggaaccaagatagcactcgaacgacgaagtaaagaacgcgaaaaagcggaaaaagcagcagagaagaaacgacgacgagaggagcagaaacagaaagataaacttaagattcgaaaactcgccttaaagccccgcagttactggattaaacaagcccaacaagccgtaaacgccttcatcagagaaagagaccgcgacttaccatgtatctcgtgcggaacgctcacgtctgctcagtgggatgccggacattaccggacaactgctgcggcacctcaactccgatttaatgaacgcaatattcacaagcaatgcgtggtgtgcaaccagcacaaaagcggaaatctcgttccgtatcgcgtcgaactgattagccgcatcgggcaggaagcagtagacgaaatcgaatcaaaccataaccgccatcgctggactatcgaagagtgcaaggcgatcaaggcagagtaccaacagaaactcaaagacctgcgaaatagcagaagtgaggccgcatgacgttctcagtaaaaaccattccagacatgctcgttgaagcatacggaaatcagacagaagtagcacgcagactgaaatgtagtcgcggtacggtcagaaaatacgttgatgataaagacgggaaaatgcacgccatcgtcaacgacgttctcatggttcatcgcggatggagtgaaagagatgcgctattacgaaaaaattgatggcagcaaataccgaaatatttgggtagttggcgatctgcacggatgctacacgaacctgatgaacaaactggatacgattggattcgacaacaaaaaagacctgcttatctcggtgggcgatttggttgatcgtggtgcagagaacgttgaatgcctggaattaatcacattcccctggttcagagctgtacgtggaaaccatgagcaaatgatgattgatggcttatcagagcgtggaaacgttaatcactggctgcttaatggcggtggctggttctttaatctcgattacgacaaagaaattctggctaaagctcttgcccataaagcagatgaacttccgttaatcatcgaactggtgagcaaagataaaaaatatgttatctgccacgccgattatccctttgacgaatacgagtttggaaagccagttgatcatcagcaggtaatctggaaccgcgaacgaatcagcaactcacaaaacgggatcgtgaaagaaatcaaaggcgcggacacgttcatctttggtcatacgccagcagtgaaaccactcaagtttgccaaccaaatgtatatcgataccggcgcagtgttctgcggaaacctaacattgattcaggtacagggagaaggcgcatgagactcgaaagcgtagctaaatttcattcgccaaaaagcccgatgatgagcgactcaccacgggccacggcttctgactctctttccggtactgatgtgatggctgctatggggatggcgcaatcacaagccggattcggtatggctgcattctgcggtaagcacgaactcagccagaacgacaaacaaaaggctatcaactatctgatgcaatttgcacacaaggtatcggggaaataccgtggtgtggcaaagcttgaaggaaatactaaggcaaaggtactgcaagtgctcgcaacattcgcttatgcggattattgccgtagtgccgcgacgccgggggcaagatgcagagattgccatggtacaggccgtgcggttgatattgccaaaacagagctgtgggggagagttgtcgagaaagagtgcggaagatgcaaaggcgtcggctattcaaggatgccagcaagcgcagcatatcgcgctgtgacgatgctaatcccaaaccttacccaacccacctggtcacgcactgttaagccgctgtatgacgctctggtggtgcaatgccacaaagaagagtcaatcgcagacaacattttgaatgcggtcacacgttagcagcatgattgccacggatggcaacatattaacggcatgatattgacttattgaataaaattgggtaaatttgactcaacgatgggttaattcgctcgttgtggtagtgagatgaaaagaggcggcgcttactaccgattccgcctagttggtcacttcgacgtatcgtctggaactccaaccatcgcaggcagagaggtctgcaaaatgcaatcccgaaacagttcgcaggtaatagttagagcctgcataacggtttcgggattttttatatctgcacaacaggtaagagcattgagtcgataatcgtgaagagtcggcgagcctggttagccagtgctctttccgttgtgctgaattaagcgaataccggaagcagaaccggatcaccaaatgcgtacaggcgtcatcgccgcccagcaacagcacaacccaaactgagccgtagccactgtctgtcctgaattcattagtaatagttacgctgcggccttttacacatgaccttcgtgaaagcgggtggcaggaggtcgcgctaacaacctcctgccgttttgcccgtgcatatcggtcacgaacaaatctgattactaaacacagtagcctggatttgttctatcagtaatcgaccttattcctaattaaatagagcaaatccccttattgggggtaagacatgaagatgccagaaaaacatgacctgttggccgccattctcgcggcaaaggaacaaggcatcggggcaatccttgcgtttgcaatggcgtaccttcgcggcagatataatggcggtgcgtttacaaaaacagtaatcgacgcaacgatgtgcgccattatcgcctggttcattcgtgaccttctcgacttcgccggactaagtagcaatctcgcttatataacgagcgtgtttatcggctacatcggtactgactcgattggttcgcttatcaaacgcttcgctgctaaaaaagccggagtagaagatggtagaaatcaataatcaacgtaaggcgttcctcgatatgctggcgtggtcggagggaactgataacggacgtcagaaaaccagaaatcatggttatgacgtcattgtaggcggagagctatttactgattactccgatcaccctcgcaaacttgtcacgctaaacccaaaactcaaatcaacaggcgccggacgctaccagcttctttcccgttggtgggatgcctaccgcaagcagcttggcctgaaagacttctctccgaaaagtcaggacgctgtggcattgcagcagattaaggagcgtggcgctttacctatgattgatcgtggtgatatccgtcaggcaatcgaccgttgcagcaatatctgggcttcactgccgggcgctggttatggtcagttcgagcataaggctgacagcctgattgcaaaattcaaagaagcgggcggaacggtcagagagattgatgtatgagcagagtcaccgcgattatctccgctctggttatctgcatcatcgtctgcctgtcatgggctgttaatcattaccgtgataacgccattacctacaaagcccagcgcgacaaaaatgccagagaactgaagctggcgaacgcggcaattactgacatgcagatgcgtcagcgtgatgttgctgcgctcgatgcaaaatacacgaaggagttagctgatgctaaagctgaaaatgatgctctgcgtgatgatgttgccgctggtcgtcgtcggttgcacatcaaagcagtctgtcagtcagtgcgtgaagccaccaccgcctccggcgtggataatgcagcctccccccgactggcagacaccgctgaacgggattatttcaccctcagagagaggctgatcactatgcaaaaacaactggaaggaacccagaagtatattaatgagcagtgcagatagagttgcccatatcgatgggcaactcatgcaattattgtgagcaatacacacgcgcttccagcggagtataaatgcctaaagtaataaaaccgagcaatccatttacgaatgtttgctgggtttctgttttaacaacattttctgcgccgccacaaattttggctgcatcgacagttttcttctgcccaattccagaaacgaagaaatgatgggtgatggtttcctttggtgctactgctgccggtttgttttgaacagtaaacgtctgttgagcacatcctgtaataagcagggccagcgcagtagcgagtagcatttttttcatggtgttattcccgatgctttttgaagttcgcagaatcgtatgtgtagaaaattaaacaaaccctaaacaatgagttgaaatttcatattgttaatatttattaatgtatgtcaggtgcgatgaatcgtcattgtattcccggattaactatgtccacagccctgacggggaacttctctgcgggagtgtccgggaataattaaaacgatgcacacagggtttagcgcgtacacgtattgcattatgccaacgccccggtgctgacacggaagaaaccggacgttatgatttagcgtggaaagatttgtgtagtgttctgaatgctctcagtaaatagtaatgaattatcaaaggtatagtaatatcttttatgttcatggatatttgtaacccatcggaaaactcctgctttagcaagattttccctgtattgctgaaatgtgatttctcttgatttcaacctatcataggacgtttctataagatgcgtgtttcttgagaatttaacatttacaacctttttaagtccttttattaacacggtgttatcgttttctaacacgatgtgaatattatctgtggctagatagtaaatataatgtgagacgttgtgacgttttagttcagaataaaacaattcacagtctaaatcttttcgcacttgatcgaatatttctttaaaaatggcaacctgagccattggtaaaaccttccatgtgatacgagggcgcgtagtttgcattatcgtttttatcgtttcaatctggtctgacctccttgtgttttgttgatgatttatgtcaaatattaggaatgttttcacttaatagtattggttgcgtaacaaagtgcggtcctgctggcattctggagggaaatacaaccgacagatgtatgtaaggccaacgtgctcaaatcttcatacagaaagatttgaagtaatattttaaccgctagatgaagagcaagcgcatggagcgacaaaatgaataaagaacaatctgctgatgatccctccgtggatctgattcgtgtaaaaaatatgcttaatagcaccatttctatgagttaccctgatgttgtaattgcatgtatagaacataaggtgtctctggaagcattcagagcaattgaggcagcgttggtgaagcacgataataatatgaaggattattccctggtggttgactgatcaccataactgctaatcattcaaactatttagtctgtgacagagccaacacgcagtctgtcactgtcaggaaagtggtaaaactgcaactcaattactgcaatgccctcgtaattaagtgaatttacaatatcgtcctgttcggagggaagaacgcgggatgttcattcttcatcacttttaattgatgtatatgctctcttttctgacgttagtctccgacggcaggcttcaatgacccaggctgagaaattcccggaccctttttgctcaagagcgatgttaatttgttcaatcatttggttaggaaagcggatgttgcgggttgttgttctgcgggttctgttcttcgttgacatgaggttgccccgtattcagtgtcgctgatttgtattgtctgaagttgtttttacgttaagttgatgcagatcaattaatacgatacctgcgtcataattgattatttgacgtggtttgatggcctccacgcacgttgtgatatgtagatgataatcattatcactttacgggtcctttccggtgatccgacaggttacg

SEQ ID NO: 37 - DNA, 32 bp, Artificial Sequence
  Anti NDM spacer (N1)
ctgagcaccgcattagccgctgcattgatgct

SEQ ID NO: 38 - DNA, 32 bp, Artificial Sequence
  Anti NDM spacer (N2)
caggagatcaacctgccggtcgcgctggcggt

SEQ ID NO: 39 - DNA, 32 bp, Artificial Sequence
  Anti NDM spacer (N3)
cgatgtcggtgccgtcgatcccaacggtgata

SEQ ID NO: 40 - DNA, 32 bp, Artificial Sequence
  Anti CTX-M-15 spacer (C1)
tgtgccgctgtatgcgcaaacggcggacgtac

SEQ ID NO: 41 - DNA, 32 bp, Artificial Sequence
  Anti CTX-M-15 spacer (C2)
ctgattgctcacgttggcggcccggctagcgt

SEQ ID NO: 42 - DNA, 32 bp, Artificial Sequence
  Anti CTX-M-15 spacer (C3)
caggcagtccagcctgaatgctcgctgcaccg

SEQ ID NO: 43 - DNA, 32 bp, Artificial Sequence
  Anti T4 Spacer (T1)
gatcgtatgctatccattacaccagcgggacg

SEQ ID NO: 44 - DNA, 32 bp, Artificial Sequence
  Anti T4 Spacer (T2)
tctgcatcacgagtacctttcatagtacgaat

SEQ ID NO: 45 - DNA, 32 bp, Artificial Sequence
  Anti T4 Spacer (T3)
cggagggcaagaaatagcttcacggtccatat

SEQ ID NO: 46 - DNA, 35 bp, Artificial Sequence
  NDM proto- spacer (N1)
aagctgagcaccgcattagccgctgcattgatgct

SEQ ID NO: 47 - DNA, 35 bp, Artificial Sequence
  NDM proto- spacer (N2)
aagcaggagatcaacctgccggtcgcgctggcggt

SEQ ID NO: 48 - DNA, 35 bp, Artificial Sequence
  NDM proto- spacer (N3)
aagcgatgtcggtgccgtcgatcccaacggtgata

SEQ ID NO: 49 - DNA, 35 bp, Artificial Sequence
  CTX-M-15 Proto-spacer (C1)
aagtgtgccgctgtatgcgcaaacggcggacgtac

SEQ ID NO: 50 - DNA, 35 bp, Artificial Sequence
  CTX-M-15 Proto-spacer (C2)
aagctgattgctcacgttggcggcccggctagcgt

SEQ ID NO: 51 - DNA, 35 bp, Artificial Sequence
  CTX-M-15 Proto-spacer (C3)
aagcaggcagtccagcctgaatgctcgctgcaccg

SEQ ID NO: 52 - DNA, 35 bp, Artificial Sequence
  T4 Proto-spacer (T1)
aaggatcgtatgctatccattacaccagcgggacg

SEQ ID NO: 53 - DNA, 35 bp, Artificial Sequence
  T4 Proto-spacer (T2)
aagtctgcatcacgagtacctttcatagtacgaat

SEQ ID NO: 54 - DNA, 35 bp, Artificial Sequence
  T4 Proto-spacer (T3)
aagcggagggcaagaaatagcttcacggtccatat

SEQ ID NO: 55 - DNA, 2022 bp, Artificial Sequence
  T7 phage with proto-spacers T7-N1N2
atgatgaacattaagactaacccgtttaaagccgtgtctttcgtagagtctgccattaagaaggctctggataacgctgggtatcttatcgctgaaatcaagtacgatggtgtacgcgggaacatctgcgtagacaatactgctaacagttactggctctctcgtgtatctaaaacgattccggcactggagcacttaaacgggtttgatgttcgctggaagcgtctactgaacgatgaccgttgcttctacaaagatggctttatgcttgatggggaactcatggtcaagggcgtagactttaacacagggtccggcctactgcgtaccaaatggactgacacgaagaaccaagagttccatgaagagttattcgttgaaccaatccgtaagaaagataaagttccctttaagctgcacactggacaccttcacataaaactgtacgctatcctcccgctgcacatcgtggagtctggagaagactgtgatgtcatgacgttgctcatgcaggaacacgttaagaacatgctgcctctgctacaggaatacttccctgaaatcgaatggcaagcggctgaatcttacgaggtctacgatatggtagaactacagcaactgtacgagcagaagcgagcagaaggccatgagggtctcattgtgaaagacccgatgtgtatctataagcgcggtaagaaatctggctggtggaaaatgaaacctgagaacgaagctgacggtatcattcagggtctggtatggggtacaaaaggtctggctaatgaaggtaaagtgattggttttgaggtgcttcttgagagtggtcgtttagttaacgccacgaatatctctcgcgccttaatggatgagttcactgagacagtaaaagaggccaccctaagtcaatggggattctttagcccatacggtattggcgacaacgatgcttgtactattaacccttacgatggctgggcgtgtcaaattagctacatggaggaaacacctgatggctctttgcggcacccatcgttcgtaatgttccgtggcaccgaggacaaccctcaagagaaaatgtaaaagctgagcaccgcattagccgctgcattgatgctgatccgtcagcctgcagttcgaagttcctatactttctagagaataggaacttcgtgtggtagaatatcagcttactattgctttacgaaagcgtatccggtgaaataaagtcaacctttagttggttaatgttacaccaacaacgaaaccaacacgccaggcttattcctgtggagttatatatgagcgataaaattattcacctgactgacgacagttttgacacggatgtactcaaagcggacggggcgatcctcgtcgatttctgggcagagtggtgcggtccgtgcaaaatgatcgccccgattctggatgaaatcgctgacgaatatcagggcaaactgaccgttgcaaaactgaacatcgatcaaaaccctggcactgcgccgaaatatggcatccgtggtatcccgactctgctgctgttcaaaaacggtgaagtggcggcaaccaaagtgggcgcactgtctaaaggtcagttgaaagagttcctcgacgctaacctggcgtaagaagttcctatactttctagagaataggaacttcgaagcagctccagcctacaaagcaggagatcaacctgccggtcgcgctggcggttcacactggctcaccttcgggtgggcctttctgcgtttataaggagacactttatgtttaagaaggttggtaaattccttgcggctttggcagctatcctgacgcttgcgtatattcttgcggtataccctcaagtagcactagtagtagttggcgcttgttacttagcggcagtgtgtgcttgcgtgtggagtatagttaactggtaatacgactcactaaaggaggtacacaccatgatgtacttaatgccattactcatcgtcattgtaggatgccttgcgctccactgtagcgatgatgata

SEQ ID NO: 56 - DNA, 2022 bp, Artificial Sequence
  T7 phage with proto-spacers T7-C2C1
atgatgaacattaagactaacccgtttaaagccgtgtctttcgtagagtctgccattaagaaggctctggataacgctgggtatcttatcgctgaaatcaagtacgatggtgtacgcgggaacatctgcgtagacaatactgctaacagttactggctctctcgtgtatctaaaacgattccggcactggagcacttaaacgggtttgatgttcgctggaagcgtctactgaacgatgaccgttgcttctacaaagatggctttatgcttgatggggaactcatggtcaagggcgtagactttaacacagggtccggcctactgcgtaccaaatggactgacacgaagaaccaagagttccatgaagagttattcgttgaaccaatccgtaagaaagataaagttccctttaagctgcacactggacaccttcacataaaactgtacgctatcctcccgctgcacatcgtggagtctggagaagactgtgatgtcatgacgttgctcatgcaggaacacgttaagaacatgctgcctctgctacaggaatacttccctgaaatcgaatggcaagcggctgaatcttacgaggtctacgatatggtagaactacagcaactgtacgagcagaagcgagcagaaggccatgagggtctcattgtgaaagacccgatgtgtatctataagcgcggtaagaaatctggctggtggaaaatgaaacctgagaacgaagctgacggtatcattcagggtctggtatggggtacaaaaggtctggctaatgaaggtaaagtgattggttttgaggtgcttcttgagagtggtcgtttagttaacgccacgaatatctctcgcgccttaatggatgagttcactgagacagtaaaagaggccaccctaagtcaatggggattctttagcccatacggtattggcgacaacgatgcttgtactattaacccttacgatggctgggcgtgtcaaattagctacatggaggaaacacctgatggctctttgcggcacccatcgttcgtaatgttccgtggcaccgaggacaaccctcaagagaaaatgtaaaagctgattgctcacgttggcggcccggctagcgtgatccgtcagcctgcagttcgaagttcctatactttctagagaataggaacttcgtgtggtagaatatcagcttactattgctttacgaaagcgtatccggtgaaataaagtcaacctttagttggttaatgttacaccaacaacgaaaccaacacgccaggcttattcctgtggagttatatatgagcgataaaattattcacctgactgacgacagttttgacacggatgtactcaaagcggacggggcgatcctcgtcgatttctgggcagagtggtgcggtccgtgcaaaatgatcgccccgattctggatgaaatcgctgacgaatatcagggcaaactgaccgttgcaaaactgaacatcgatcaaaaccctggcactgcgccgaaatatggcatccgtggtatcccgactctgctgctgttcaaaaacggtgaagtggcggcaaccaaagtgggcgcactgtctaaaggtcagttgaaagagttcctcgacgctaacctggcgtaagaagttcctatactttctagagaataggaacttcgaagcagctccagcctacaaagtgtgccgctgtatgcgcaaacggcggacgtactcacactggctcaccttcgggtgggcctttctgcgtttataaggagacactttatgtttaagaaggttggtaaattccttgcggctttggcagctatcctgacgcttgcgtatattcttgcggtataccctcaagtagcactagtagtagttggcgcttgttacttagcggcagtgtgtgcttgcgtgtggagtatagttaactggtaatacgactcactaaaggaggtacacaccatgatgtacttaatgccattactcatcgtcattgtaggatgccttgcgctccactgtagcgatgatgata

SEQ ID NO: 57 - DNA, 2022 bp, Artificial Sequence
  T7 phage with proto-spacers T7N1C1
atgatgaacattaagactaacccgtttaaagccgtgtctttcgtagagtctgccattaagaaggctctggataacgctgggtatcttatcgctgaaatcaagtacgatggtgtacgcgggaacatctgcgtagacaatactgctaacagttactggctctctcgtgtatctaaaacgattccggcactggagcacttaaacgggtttgatgttcgctggaagcgtctactgaacgatgaccgttgcttctacaaagatggctttatgcttgatggggaactcatggtcaagggcgtagactttaacacagggtccggcctactgcgtaccaaatggactgacacgaagaaccaagagttccatgaagagttattcgttgaaccaatccgtaagaaagataaagttccctttaagctgcacactggacaccttcacataaaactgtacgctatcctcccgctgcacatcgtggagtctggagaagactgtgatgtcatgacgttgctcatgcaggaacacgttaagaacatgctgcctctgctacaggaatacttccctgaaatcgaatggcaagcggctgaatcttacgaggtctacgatatggtagaactacagcaactgtacgagcagaagcgagcagaaggccatgagggtctcattgtgaaagacccgatgtgtatctataagcgcggtaagaaatctggctggtggaaaatgaaacctgagaacgaagctgacggtatcattcagggtctggtatggggtacaaaaggtctggctaatgaaggtaaagtgattggttttgaggtgcttcttgagagtggtcgtttagttaacgccacgaatatctctcgcgccttaatggatgagttcactgagacagtaaaagaggccaccctaagtcaatggggattctttagcccatacggtattggcgacaacgatgcttgtactattaacccttacgatggctgggcgtgtcaaattagctacatggaggaaacacctgatggctctttgcggcacccatcgttcgtaatgttccgtggcaccgaggacaaccctcaagagaaaatgtaaaagctgagcaccgcattagccgctgcattgatgctgatccgtcagcctgcagttcgaagttcctatactttctagagaataggaacttcgtgtggtagaatatcagcttactattgctttacgaaagcgtatccggtgaaataaagtcaacctttagttggttaatgttacaccaacaacgaaaccaacacgccaggcttattcctgtggagttatatatgagcgataaaattattcacctgactgacgacagttttgacacggatgtactcaaagcggacggggcgatcctcgtcgatttctgggcagagtggtgcggtccgtgcaaaatgatcgccccgattctggatgaaatcgctgacgaatatcagggcaaactgaccgttgcaaaactgaacatcgatcaaaaccctggcactgcgccgaaatatggcatccgtggtatcccgactctgctgctgttcaaaaacggtgaagtggcggcaaccaaagtgggcgcactgtctaaaggtcagttgaaagagttcctcgacgctaacctggcgtaagaagttcctatactttctagagaataggaacttcgaagcagctccagcctacaaagtgtgccgctgtatgcgcaaacggcggacgtactcacactggctcaccttcgggtgggcctttctgcgtttataaggagacactttatgtttaagaaggttggtaaattccttgcggctttggcagctatcctgacgcttgcgtatattcttgcggtataccctcaagtagcactagtagtagttggcgcttgttacttagcggcagtgtgtgcttgcgtgtggagtatagttaactggtaatacgactcactaaaggaggtacacaccatgatgtacttaatgccattactcatcgtcattgtaggatgccttgcgctccactgtagcgatgatgata

SEQ ID NO: 58 - DNA, 2022 bp, Artificial Sequence
  T7 phage with proto-spacers T7-C2N2
atgatgaacattaagactaacccgtttaaagccgtgtctttcgtagagtctgccattaagaaggctctggataacgctgggtatcttatcgctgaaatcaagtacgatggtgtacgcgggaacatctgcgtagacaatactgctaacagttactggctctctcgtgtatctaaaacgattccggcactggagcacttaaacgggtttgatgttcgctggaagcgtctactgaacgatgaccgttgcttctacaaagatggctttatgcttgatggggaactcatggtcaagggcgtagactttaacacagggtccggcctactgcgtaccaaatggactgacacgaagaaccaagagttccatgaagagttattcgttgaaccaatccgtaagaaagataaagttccctttaagctgcacactggacaccttcacataaaactgtacgctatcctcccgctgcacatcgtggagtctggagaagactgtgatgtcatgacgttgctcatgcaggaacacgttaagaacatgctgcctctgctacaggaatacttccctgaaatcgaatggcaagcggctgaatcttacgaggtctacgatatggtagaactacagcaactgtacgagcagaagcgagcagaaggccatgagggtctcattgtgaaagacccgatgtgtatctataagcgcggtaagaaatctggctggtggaaaatgaaacctgagaacgaagctgacggtatcattcagggtctggtatggggtacaaaaggtctggctaatgaaggtaaagtgattggttttgaggtgcttcttgagagtggtcgtttagttaacgccacgaatatctctcgcgccttaatggatgagttcactgagacagtaaaagaggccaccctaagtcaatggggattctttagcccatacggtattggcgacaacgatgcttgtactattaacccttacgatggctgggcgtgtcaaattagctacatggaggaaacacctgatggctctttgcggcacccatcgttcgtaatgttccgtggcaccgaggacaaccctcaagagaaaatgtaaaagctgattgctcacgttggcggcccggctagcgtgatccgtcagcctgcagttcgaagttcctatactttctagagaataggaacttcgtgtggtagaatatcagcttactattgctttacgaaagcgtatccggtgaaataaagtcaacctttagttggttaatgttacaccaacaacgaaaccaacacgccaggcttattcctgtggagttatatatgagcgataaaattattcacctgactgacgacagttttgacacggatgtactcaaagcggacggggcgatcctcgtcgatttctgggcagagtggtgcggtccgtgcaaaatgatcgccccgattctggatgaaatcgctgacgaatatcagggcaaactgaccgttgcaaaactgaacatcgatcaaaaccctggcactgcgccgaaatatggcatccgtggtatcccgactctgctgctgttcaaaaacggtgaagtggcggcaaccaaagtgggcgcactgtctaaaggtcagttgaaagagttcctcgacgctaacctggcgtaagaagttcctatactttctagagaataggaacttcgaagcagctccagcctacaaagcaggagatcaacctgccggtcgcgctggcggttcacactggctcaccttcgggtgggcctttctgcgtttataaggagacactttatgtttaagaaggttggtaaattccttgcggctttggcagctatcctgacgcttgcgtatattcttgcggtataccctcaagtagcactagtagtagttggcgcttgttacttagcggcagtgtgtgcttgcgtgtggagtatagttaactggtaatacgactcactaaaggaggtacacaccatgatgtacttaatgccattactcatcgtcattgtaggatgccttgcgctccactgtagcgatgatgata

SEQ ID NO: 59 - DNA, 48528 bp, Artificial Sequence
  Recombinant  lambda phage with the cas proteins and CRISPR array IYMMPh3
gggcggcgacctcgcgggttttcgctatttatgaaaattttccggtttaaggcgtttccgttcttcttcgtcataacttaatgtttttatttaaaataccctctgaaaagaaaggaaacgacaggtgctgaaagcgaggctttttggcctctgtcgtttcctttctctgtttttgtccgtggaatgaacaatggaagtcaacaaaaagcagctggctgacattttcggtgcgagtatccgtaccattcagaactggcaggaacagggaatgcccgttctgcgaggcggtggcaagggtaatgaggtgctttatgactctgccgccgtcataaaatggtatgccgaaagggatgctgaaattgagaacgaaaagctgcgccgggaggttgaagaactgcggcaggccagcgaggcagatctccagccaggaactattgagtacgaacgccatcgacttacgcgtgcgcaggccgacgcacaggaactgaagaatgccagagactccgctgaagtggtggaaaccgcattctgtactttcgtgctgtcgcggatcgcaggtgaaattgccagtattctcgacgggctccccctgtcggtgcagcggcgttttccggaactggaaaaccgacatgttgatttcctgaaacgggatatcatcaaagccatgaacaaagcagccgcgctggatgaactgataccggggttgctgagtgaatatatcgaacagtcaggttaacaggctgcggcattttgtccgcgccgggcttcgctcactgttcaggccggagccacagaccgccgttgaatgggcggatgctaattactatctcccgaaagaatccgcataccaggaagggcgctgggaaacactgccctttcagcgggccatcatgaatgcgatgggcagcgactacatccgtgaggtgaatgtggtgaagtctgcccgtgtcggttattccaaaatgctgctgggtgtttatgcctactttatagagcataagcagcgcaacacccttatctggttgccgacggatggtgatgccgagaactttatgaaaacccacgttgagccgactattcgtgatattccgtcgctgctggcgctggccccgtggtatggcaaaaagcaccgggataacacgctcaccatgaagcgtttcactaatgggcgtggcttctggtgcctgggcggtaaagcggcaaaaaactaccgtgaaaagtcggtggatgtggcgggttatgatgaacttgctgcttttgatgatgatattgaacaggaaggctctccgacgttcctgggtgacaagcgtattgaaggctcggtctggccaaagtccatccgtggctccacgccaaaagtgagaggcacctgtcagattgagcgtgcagccagtgaatccccgcattttatgcgttttcatgttgcctgcccgcattgcggggaggagcagtatcttaaatttggcgacaaagagacgccgtttggcctcaaatggacgccggatgacccctccagcgtgttttatctctgcgagcataatgcctgcgtcatccgccagcaggagctggactttactgatgcccgttatatctgcgaaaagaccgggatctggacccgtgatggcattctctggttttcgtcatccggtgaagagattgagccacctgacagtgtgacctttcacatctggacagcgtacagcccgttcaccacctgggtgcagattgtcaaagactggatgaaaacgaaaggggatacgggaaaacgtaaaaccttcgtaaacaccacgctcggtgagacgtgggaggcgaaaattggcgaacgtccggatgctgaagtgatggcagagcggaaagagcattattcagcgcccgttcctgaccgtgtggcttacctgaccgccggtatcgactcccagctggaccgctacgaaatgcgcgtatggggatgggggccgggtgaggaaagctggctgattgaccggcagattattatgggccgccacgacgatgaacagacgctgctgcgtgtggatgaggccatcaataaaacctatacccgccggaatggtgcagaaatgtcgatatcccgtatctgctgggatactggcgggattgacccgaccattgtgtatgaacgctcgaaaaaacatgggctgttccgggtgatccccattaaaggggcatccgtctacggaaagccggtggccagcatgccacgtaagcgaaacaaaaacggggtttaccttaccgaaatcggtacggataccgcgaaagagcagatttataaccgcttcacactgacgccggaaggggatgaaccgcttcccggtgccgttcacttcccgaataacccggatatttttgatctgaccgaagcgcagcagctgactgctgaagagcaggtcgaaaaatgggtggatggcaggaaaaaaatactgtgggacagcaaaaagcgacgcaatgaggcactcgactgcttcgtttatgcgctggcggcgctgcgcatcagtatttcccgctggcagctggatctcagtgcgctgctggcgagcctgcaggaagaggatggtgcagcaaccaacaagaaaacactggcagattacgcccgtgccttatccggagaggatgaatgacgcgacaggaagaacttgccgctgcccgtgcggcactgcatgacctgatgacaggtaaacgggtggcaacagtacagaaagacggacgaagggtggagtttacggccacttccgtgtctgacctgaaaaaatatattgcagagctggaagtgcagaccggcatgacacagcgacgcaggggacctgcaggattttatgtatgaaaacgcccaccattcccacccttctggggccggacggcatgacatcgctgcgcgaatatgccggttatcacggcggtggcagcggatttggagggcagttgcggtcgtggaacccaccgagtgaaagtgtggatgcagccctgttgcccaactttacccgtggcaatgcccgcgcagacgatctggtacgcaataacggctatgccgccaacgccatccagctgcatcaggatcatatcgtcgggtcttttttccggctcagtcatcgcccaagctggcgctatctgggcatcggggaggaagaagcccgtgccttttcccgcgaggttgaagcggcatggaaagagtttgccgaggatgactgctgctgcattgacgttgagcgaaaacgcacgtttaccatgatgattcgggaaggtgtggccatgcacgcctttaacggtgaactgttcgttcaggccacctgggataccagttcgtcgcggcttttccggacacagttccggatggtcagcccgaagcgcatcagcaacccgaacaataccggcgacagccggaactgccgtgccggtgtgcagattaatgacagcggtgcggcgctgggatattacgtcagcgaggacgggtatcctggctggatgccgcagaaatggacatggataccccgtgagttacccggcgggcgcgcctcgttcattcacgtttttgaacccgtggaggacgggcagactcgcggtgcaaatgtgttttacagcgtgatggagcagatgaagatgctcgacacgctgcagaacacgcagctgcagagcgccattgtgaaggcgatgtatgccgccaccattgagagtgagctggatacgcagtcagcgatggattttattctgggcgcgaacagtcaggagcagcgggaaaggctgaccggctggattggtgaaattgccgcgtattacgccgcagcgccggtccggctgggaggcgcaaaagtaccgcacctgatgccgggtgactcactgaacctgcagacggctcaggatacggataacggctactccgtgtttgagcagtcactgctgcggtatatcgctgccgggctgggtgtctcgtatgagcagctttcccggaattacgcccagatgagctactccacggcacgggccagtgcgaacgagtcgtgggcgtactttatggggcggcgaaaattcgtcgcatcccgtcaggcgagccagatgtttctgtgctggctggaagaggccatcgttcgccgcgtggtgacgttaccttcaaaagcgcgcttcagttttcaggaagcccgcagtgcctgggggaactgcgactggataggctccggtcgtatggccatcgatggtctgaaagaagttcaggaagcggtgatgctgatagaagccggactgagtacctacgagaaagagtgcgcaaaacgcggtgacgactatcaggaaatttttgcccagcaggtccgtgaaacgatggagcgccgtgcagccggtcttaaaccgcccgcctgggcggctgcagcatttgaatccgggctgcgacaatcaacagaggaggagaagagtgacagcagagctgcgtaatctcccgcatattgccagcatggcctttaatgagccgctgatgcttgaacccgcctatgcgcgggttttcttttgtgcgcttgcaggccagcttgggatcagcagcctgacggatgcggtgtccggcgacagcctgactgcccaggaggcactcgcgacgctggcattatccggtgatgatgacggaccacgacaggcccgcagttatcaggtcatgaacggcatcgccgtgctgccggtgtccggcacgctggtcagccggacgcgggcgctgcagccgtactcggggatgaccggttacaacggcattatcgcccgtctgcaacaggctgccagcgatccgatggtggacggcattctgctcgatatggacacgcccggcgggatggtggcgggggcatttgactgcgctgacatcatcgcccgtgtgcgtgacataaaaccggtatgggcgcttgccaacgacatgaactgcagtgcaggtcagttgcttgccagtgccgcctcccggcgtctggtcacgcagaccgcccggacaggctccatcggcgtcatgatggctcacagtaattacggtgctgcgctggagaaacagggtgtggaaatcacgctgatttacagcggcagccataaggtggatggcaacccctacagccatcttccggatgacgtccgggagacactgcagtcccggatggacgcaacccgccagatgtttgcgcagaaggtgtcggcatataccggcctgtccgtgcaggttgtgctggataccgaggctgcagtgtacagcggtcaggaggccattgatgccggactggctgatgaacttgttaacagcaccgatgcgatcaccgtcatgcgtgatgcactggatgcacgtaaatcccgtctctcaggagggcgaatgaccaaagagactcaatcaacaactgtttcagccactgcttcgcaggctgacgttactgacgtggtgccagcgacggagggcgagaacgccagcgcggcgcagccggacgtgaacgcgcagatcaccgcagcggttgcggcagaaaacagccgcattatggggatcctcaactgtgaggaggctcacggacgcgaagaacaggcacgcgtgctggcagaaacccccggtatgaccgtgaaaacggcccgccgcattctggccgcagcaccacagagtgcacaggcgcgcagtgacactgcgctggatcgtctgatgcagggggcaccggcaccgctggctgcaggtaacccggcatctgatgccgttaacgatttgctgaacacaccagtgtaagggatgtttatgacgagcaaagaaacctttacccattaccagccgcagggcaacagtgacccggctcataccgcaaccgcgcccggcggattgagtgcgaaagcgcctgcaatgaccccgctgatgctggacacctccagccgtaagctggttgcgtgggatggcaccaccgacggtgctgccgttggcattcttgcggttgctgctgaccagaccagcaccacgctgacgttctacaagtccggcacgttccgttatgaggatgtgctctggccggaggctgccagcgacgagacgaaaaaacggaccgcgtttgccggaacggcaatcagcatcgtttaactttacccttcatcactaaaggccgcctgtgcggctttttttacgggatttttttatgtcgatgtacacaaccgcccaactgctggcggcaaatgagcagaaatttaagtttgatccgctgtttctgcgtctctttttccgtgagagctatcccttcaccacggagaaagtctatctctcacaaattccgggactggtaaacatggcgctgtacgtttcgccgattgtttccggtgaggttatccgttcccgtggcggctccacctctgaatttacgccgggatatgtcaagccgaagcatgaagtgaatccgcagatgaccctgcgtcgcctgccggatgaagatccgcagaatctggcggacccggcttaccgccgccgtcgcatcatcatgcagaacatgcgtgacgaagagctggccattgctcaggtcgaagagatgcaggcagtttctgccgtgcttaagggcaaatacaccatgaccggtgaagccttcgatccggttgaggtggatatgggccgcagtgaggagaataacatcacgcagtccggcggcacggagtggagcaagcgtgacaagtccacgtatgacccgaccgacgatatcgaagcctacgcgctgaacgccagcggtgtggtgaatatcatcgtgttcgatccgaaaggctgggcgctgttccgttccttcaaagccgtcaaggagaagctggatacccgtcgtggctctaattccgagctggagacagcggtgaaagacctgggcaaagcggtgtcctataaggggatgtatggcgatgtggccatcgtcgtgtattccggacagtacgtggaaaacggcgtcaaaaagaacttcctgccggacaacacgatggtgctggggaacactcaggcacgcggtctgcgcacctatggctgcattcaggatgcggacgcacagcgcgaaggcattaacgcctctgcccgttacccgaaaaactgggtgaccaccggcgatccggcgcgtgagttcaccatgattcagtcagcaccgctgatgctgctggctgaccctgatgagttcgtgtccgtacaactggcgtaatcatggcccttcggggccattgtttctctgtggaggagtccatgacgaaagatgaactgattgcccgtctccgctcgctgggtgaacaactgaaccgtgatgtcagcctgacggggacgaaagaagaactggcgctccgtgtggcagagctgaaagaggagcttgatgacacggatgaaactgccggtcaggacacccctctcagccgggaaaatgtgctgaccggacatgaaaatgaggtgggatcagcgcagccggataccgtgattctggatacgtctgaactggtcacggtcgtggcactggtgaagctgcatactgatgcacttcacgccacgcgggatgaacctgtggcatttgtgctgccgggaacggcgtttcgtgtctctgccggtgtggcagccgaaatgacagagcgcggcctggccagaatgcaataacgggaggcgctgtggctgatttcgataacctgttcgatgctgccattgcccgcgccgatgaaacgatacgcgggtacatgggaacgtcagccaccattacatccggtgagcagtcaggtgcggtgatacgtggtgtttttgatgaccctgaaaatatcagctatgccggacagggcgtgcgcgttgaaggctccagcccgtccctgtttgtccggactgatgaggtgcggcagctgcggcgtggagacacgctgaccatcggtgaggaaaatttctgggtagatcgggtttcgccggatgatggcggaagttgtcatctctggcttggacggggcgtaccgcctgccgttaaccgtcgccgctgaaagggggatgtatggccataaaaggtcttgagcaggccgttgaaaacctcagccgtatcagcaaaacggcggtgcctggtgccgccgcaatggccattaaccgcgttgcttcatccgcgatatcgcagtcggcgtcacaggttgcccgtgagacaaaggtacgccggaaactggtaaaggaaagggccaggctgaaaagggccacggtcaaaaatccgcaggccagaatcaaagttaaccggggggatttgcccgtaatcaagctgggtaatgcgcgggttgtcctttcgcgccgcaggcgtcgtaaaaaggggcagcgttcatccctgaaaggtggcggcagcgtgcttgtggtgggtaaccgtcgtattcccggcgcgtttattcagcaactgaaaaatggccggtggcatgtcatgcagcgtgtggctgggaaaaaccgttaccccattgatgtggtgaaaatcccgatggcggtgccgctgaccacggcgtttaaacaaaatattgagcggatacggcgtgaacgtcttccgaaagagctgggctatgcgctgcagcatcaactgaggatggtaataaagcgatgaaacatactgaactccgtgcagccgtactggatgcactggagaagcatgacaccggggcgacgttttttgatggtcgccccgctgtttttgatgaggcggattttccggcagttgccgtttatctcaccggcgctgaatacacgggcgaagagctggacagcgatacctggcaggcggagctgcatatcgaagttttcctgcctgctcaggtgccggattcagagctggatgcgtggatggagtcccggatttatccggtgatgagcgatatcccggcactgtcagatttgatcaccagtatggtggccagcggctatgactaccggcgcgacgatgatgcgggcttgtggagttcagccgatctgacttatgtcattacctatgaaatgtgaggacgctatgcctgtaccaaatcctacaatgccggtgaaaggtgccgggaccaccctgtgggtttataaggggagcggtgacccttacgcgaatccgctttcagacgttgactggtcgcgtctggcaaaagttaaagacctgacgcccggcgaactgaccgctgagtcctatgacgacagctatctcgatgatgaagatgcagactggactgcgaccgggcaggggcagaaatctgccggagataccagcttcacgctggcgtggatgcccggagagcaggggcagcaggcgctgctggcgtggtttaatgaaggcgatacccgtgcctataaaatccgcttcccgaacggcacggtcgatgtgttccgtggctgggtcagcagtatcggtaaggcggtgacggcgaaggaagtgatcacccgcacggtgaaagtcaccaatgtgggacgtccgtcgatggcagaagatcgcagcacggtaacagcggcaaccggcatgaccgtgacgcctgccagcacctcggtggtgaaagggcagagcaccacgctgaccgtggccttccagccggagggcgtaaccgacaagagctttcgtgcggtgtctgcggataaaacaaaagccaccgtgtcggtcagtggtatgaccatcaccgtgaacggcgttgctgcaggcaaggtcaacattccggttgtatccggtaatggtgagtttgctgcggttgcagaaattaccgtcaccgccagttaatccggagagtcagcgatgttcctgaaaaccgaatcatttgaacataacggtgtgaccgtcacgctttctgaactgtcagccctgcagcgcattgagcatctcgccctgatgaaacggcaggcagaacaggcggagtcagacagcaaccggaagtttactgtggaagacgccatcagaaccggcgcgtttctggtggcgatgtccctgtggcataaccatccgcagaagacgcagatgccgtccatgaatgaagccgttaaacagattgagcaggaagtgcttaccacctggcccacggaggcaatttctcatgctgaaaacgtggtgtaccggctgtctggtatgtatgagtttgtggtgaataatgcccctgaacagacagaggacgccgggcccgcagagcctgtttctgcgggaaagtgttcgacggtgagctgagttttgccctgaaactggcgcgtgagatggggcgacccgactggcgtgccatgcttgccgggatgtcatccacggagtatgccgactggcaccgcttttacagtacccattattttcatgatgttctgctggatatgcacttttccgggctgacgtacaccgtgctcagcctgtttttcagcgatccggatatgcatccgctggatttcagtctgctgaaccggcgcgaggctgacgaagagcctgaagatgatgtgctgatgcagaaagcggcagggcttgccggaggtgtccgctttggcccggacgggaatgaagttatccccgcttccccggatgtggcggacatgacggaggatgacgtaatgctgatgacagtatcagaagggatcgcaggaggagtccggtatggctgaaccggtaggcgatctggtcgttgatttgagtctggatgcggccagatttgacgagcagatggccagagtcaggcgtcatttttctggtacggaaagtgatgcgaaaaaaacagcggcagtcgttgaacagtcgctgagccgacaggcgctggctgcacagaaagcggggatttccgtcgggcagtataaagccgccatgcgtatgctgcctgcacagttcaccgacgtggccacgcagcttgcaggcgggcaaagtccgtggctgatcctgctgcaacagggggggcaggtgaaggactccttcggcgggatgatccccatgttcagggggcttgccggtgcgatcaccctgccgatggtgggggccacctcgctggcggtggcgaccggtgcgctggcgtatgcctggtatcagggcaactcaaccctgtccgatttcaacaaaacgctggtcctttccggcaatcaggcgggactgacggcagatcgtatgctggtcctgtccagagccgggcaggcggcagggctgacgtttaaccagaccagcgagtcactcagcgcactggttaaggcgggggtaagcggtgaggctcagattgcgtccatcagccagagtgtggcgcgtttctcctctgcatccggcgtggaggtggacaaggtcgctgaagccttcgggaagctgaccacagacccgacgtcggggctgacggcgatggctcgccagttccataacgtgtcggcggagcagattgcgtatgttgctcagttgcagcgttccggcgatgaagccggggcattgcaggcggcgaacgaggccgcaacgaaagggtttgatgaccagacccgccgcctgaaagagaacatgggcacgctggagacctgggcagacaggactgcgcgggcattcaaatccatgtgggatgcggtgctggatattggtcgtcctgataccgcgcaggagatgctgattaaggcagaggctgcgtataagaaagcagacgacatctggaatctgcgcaaggatgattattttgttaacgatgaagcgcgggcgcgttactgggatgatcgtgaaaaggcccgtcttgcgcttgaagccgcccgaaagaaggctgagcagcagactcaacaggacaaaaatgcgcagcagcagagcgataccgaagcgtcacggctgaaatataccgaagaggcgcagaaggcttacgaacggctgcagacgccgctggagaaatataccgcccgtcaggaagaactgaacaaggcactgaaagacgggaaaatcctgcaggcggattacaacacgctgatggcggcggcgaaaaaggattatgaagcgacgctgaaaaagccgaaacagtccagcgtgaaggtgtctgcgggcgatcgtcaggaagacagtgctcatgctgccctgctgacgcttcaggcagaactccggacgctggagaagcatgccggagcaaatgagaaaatcagccagcagcgccgggatttgtggaaggcggagagtcagttcgcggtactggaggaggcggcgcaacgtcgccagctgtctgcacaggagaaatccctgctggcgcataaagatgagacgctggagtacaaacgccagctggctgcacttggcgacaaggttacgtatcaggagcgcctgaacgcgctggcgcagcaggcggataaattcgcacagcagcaacgggcaaaacgggccgccattgatgcgaaaagccgggggctgactgaccggcaggcagaacgggaagccacggaacagcgcctgaaggaacagtatggcgataatccgctggcgctgaataacgtcatgtcagagcagaaaaagacctgggcggctgaagaccagcttcgcgggaactggatggcaggcctgaagtccggctggagtgagtgggaagagagcgccacggacagtatgtcgcaggtaaaaagtgcagccacgcagacctttgatggtattgcacagaatatggcggcgatgctgaccggcagtgagcagaactggcgcagcttcacccgttccgtgctgtccatgatgacagaaattctgcttaagcaggcaatggtggggattgtcgggagtatcggcagcgccattggcggggctgttggtggcggcgcatccgcgtcaggcggtacagccattcaggccgctgcggcgaaattccattttgcaaccggaggatttacgggaaccggcggcaaatatgagccagcggggattgttcaccgtggtgagtttgtcttcacgaaggaggcaaccagccggattggcgtggggaatctttaccggctgatgcgcggctatgccaccggcggttatgtcggtacaccgggcagcatggcagacagccggtcgcaggcgtccgggacgtttgagcagaataaccatgtggtgattaacaacgacggcacgaacgggcagataggtccggctgctctgaaggcggtgtatgacatggcccgcaagggtgcccgtgatgaaattcagacacagatgcgtgatggtggcctgttctccggaggtggacgatgaagaccttccgctggaaagtgaaacccggtatggatgtggcttcggtcccttctgtaagaaaggtgcgctttggtgatggctattctcagcgagcgcctgccgggctgaatgccaacctgaaaacgtacagcgtgacgctttctgtcccccgtgaggaggccacggtactggagtcgtttctggaagagcacgggggctggaaatcctttctgtggacgccgccttatgagtggcggcagataaaggtgacctgcgcaaaatggtcgtcgcgggtcagtatgctgcgtgttgagttcagcgcagagtttgaacaggtggtgaactgatgcaggatatccggcaggaaacactgaatgaatgcacccgtgcggagcagtcggccagcgtggtgctctgggaaatcgacctgacagaggtcggtggagaacgttattttttctgtaatgagcagaacgaaaaaggtgagccggtcacctggcaggggcgacagtatcagccgtatcccattcaggggagcggttttgaactgaatggcaaaggcaccagtacgcgccccacgctgacggtttctaacctgtacggtatggtcaccgggatggcggaagatatgcagagtctggtcggcggaacggtggtccggcgtaaggtttacgcccgttttctggatgcggtgaacttcgtcaacggaaacagttacgccgatccggagcaggaggtgatcagccgctggcgcattgagcagtgcagcgaactgagcgcggtgagtgcctcctttgtactgtccacgccgacggaaacggatggcgctgtttttccgggacgtatcatgctggccaacacctgcacctggacctatcgcggtgacgagtgcggttatagcggtccggctgtcgcggatgaatatgaccagccaacgtccgatatcacgaaggataaatgcagcaaatgcctgagcggttgtaagttccgcaataacgtcggcaactttggcggcttcctttccattaacaaactttcgcagtaaatcccatgacacagacagaatcagcgattctggcgcacgcccggcgatgtgcgccagcggagtcgtgcggcttcgtggtaagcacgccggagggggaaagatatttcccctgcgtgaatatctccggtgagccggaggctatttccgtatgtcgccggaagactggctgcaggcagaaatgcagggtgagattgtggcgctggtccacagccaccccggtggtctgccctggctgagtgaggccgaccggcggctgcaggtgcagagtgatttgccgtggtggctggtctgccgggggacgattcataagttccgctgtgtgccgcatctcaccgggcggcgctttgagcacggtgtgacggactgttacacactgttccgggatgcttatcatctggcggggattgagatgccggactttcatcgtgaggatgactggtggcgtaacggccagaatctctatctggataatctggaggcgacggggctgtatcaggtgccgttgtcagcggcacagccgggcgatgtgctgctgtgctgttttggttcatcagtgccgaatcacgccgcaatttactgcggcgacggcgagctgctgcaccatattcctgaacaactgagcaaacgagagaggtacaccgacaaatggcagcgacgcacacactccctctggcgtcaccgggcatggcgcgcatctgcctttacggggatttacaacgatttggtcgccgcatcgaccttcgtgtgaaaacgggggctgaagccatccgggcactggccacacagctcccggcgtttcgtcagaaactgagcgacggctggtatcaggtacggattgccgggcgggacgtcagcacgtccgggttaacggcgcagttacatgagactctgcctgatggcgctgtaattcatattgttcccagagtcgccggggccaagtcaggtggcgtattccagattgtcctgggggctgccgccattgccggatcattctttaccgccggagccacccttgcagcatggggggcagccattggggccggtggtatgaccggcatcctgttttctctcggtgccagtatggtgctcggtggtgtggcgcagatgctggcaccgaaagccagaactccccgtatacagacaacggataacggtaagcagaacacctatttctcctcactggataacatggttgcccagggcaatgttctgcctgttctgtacggggaaatgcgcgtggggtcacgcgtggtttctcaggagatcagcacggcagacgaaggggacggtggtcaggttgtggtgattggtcgctgatgcaaaatgttttatgtgaaaccgcctgcgggcggttttgtcatttatggagcgtgaggaatgggtaaaggaagcagtaaggggcataccccgcgcgaagcgaaggacaacctgaagtccacgcagttgctgagtgtgatcgatgccatcagcgaagggccgattgaaggtccggtggatggcttaaaaagcgtgctgctgaacagtacgccggtgctggacactgaggggaataccaacatatccggtgtcacggtggtgttccgggctggtgagcaggagcagactccgccggagggatttgaatcctccggctccgagacggtgctgggtacggaagtgaaatatgacacgccgatcacccgcaccattacgtctgcaaacatcgaccgtctgcgctttaccttcggtgtacaggcactggtggaaaccacctcaaagggtgacaggaatccgtcggaagtccgcctgctggttcagatacaacgtaacggtggctgggtgacggaaaaagacatcaccattaagggcaaaaccacctcgcagtatctggcctcggtggtgatgggtaacctgccgccgcgcccgtttaatatccggatgcgcaggatgacgccggacagcaccacagaccagctgcagaacaaaacgctctggtcgtcatacactgaaatcatcgatgtgaaacagtgctacccgaacacggcactggtcggcgtgcaggtggactcggagcagttcggcagccagcaggtgagccgtaattatcatctgcgcgggcgtattctgcaggtgccgtcgaactataacccgcagacgcggcaatacagcggtatctgggacggaacgtttaaaccggcatacagcaacaacatggcctggtgtctgtgggatatgctgacccatccgcgctacggcatggggaaacgtcttggtgcggcggatgtggataaatgggcgctgtatgtcatcggccagtactgcgaccagtcagtgccggacggctttggcggcacggagccgcgcatcacctgtaatgcgtacctgaccacacagcgtaaggcgtgggatgtgctcagcgatttctgctcggcgatgcgctgtatgccggtatggaacgggcagacgctgacgttcgtgcaggaccgaccgtcggataagacgtggacctataaccgcagtaatgtggtgatgccggatgatggcgcgccgttccgctacagcttcagcgccctgaaggaccgccataatgccgttgaggtgaactggattgacccgaacaacggctgggagacggcgacagagcttgttgaagatacgcaggccattgcccgttacggtcgtaatgttacgaagatggatgcctttggctgtaccagccgggggcaggcacaccgcgccgggctgtggctgattaaaacagaactgctggaaacgcagaccgtggatttcagcgtcggcgcagaagggcttcgccatgtaccgggcgatgttattgaaatctgcgatgatgactatgccggtatcagcaccggtggtcgtgtgctggcggtgaacagccagacccggacgctgacgctcgaccgtgaaatcacgctgccatcctccggtaccgcgctgataagcctggttgacggaagtggcaatccggtcagcgtggaggttcagtccgtcaccgacggcgtgaaggtaaaagtgagccgtgttcctgacggtgttgctgaatacagcgtatgggagctgaagctgccgacgctgcgccagcgactgttccgctgcgtgagtatccgtgagaacgacgacggcacgtatgccatcaccgccgtgcagcatgtgccggaaaaagaggccatcgtggataacggggcgcactttgacggcgaacagagtggcacggtgaatggtgtcacgccgccagcggtgcagcacctgaccgcagaagtcactgcagacagcggggaatatcaggtgctggcgcgatgggacacaccgaaggtggtgaagggcgtgagtttcctgctccgtctgaccgtaacagcggacgacggcagtgagcggctggtcagcacggcccggacgacggaaaccacataccgcttcacgcaactggcgctggggaactacaggctgacagtccgggcggtaaatgcgtgggggcagcagggcgatccggcgtcggtatcgttccggattgccgcaccggcagcaccgtcgaggattgagctgacgccgggctattttcagataaccgccacgccgcatcttgccgtttatgacccgacggtacagtttgagttctggttctcggaaaagcagattgcggatatcagacaggttgaaaccagcacgcgttatcttggtacggcgctgtactggatagccgccagtatcaatatcaaaccgggccatgattattacttttatatccgcagtgtgaacaccgttggcaaatcggcattcgtggaggccgtcggtcgggcgagcgatgatgcggaaggttacctggattttttcaaaggcaagataaccgaatcccatctcggcaaggagctgctggaaaaagtcgagctgacggaggataacgccagcagactggaggagttttcgaaagagtggaaggatgccagtgataagtggaatgccatgtgggctgtcaaaattgagcagaccaaagacggcaaacattatgtcgcgggtattggcctcagcatggaggacacggaggaaggcaaactgagccagtttctggttgccgccaatcgtatcgcatttattgacccggcaaacgggaatgaaacgccgatgtttgtggcgcagggcaaccagatattcatgaacgacgtgttcctgaagcgcctgacggcccccaccattaccagcggcggcaatcctccggccttttccctgacaccggacggaaagctgaccgctaaaaatgcggatatcagtggcagtgtgaatgcgaactccgggacgctcagtaatgtgacgatagctgaaaactgtacgataaacggtacgctgagggcggaaaaaatcgtcggggacattgtaaaggcggcgagcgcggcttttccgcgccagcgtgaaagcagtgtggactggccgtcaggtacccgtactgtcaccgtgaccgatgaccatccttttgatcgccagatagtggtgcttccgctgacgtttcgcggaagtaagcgtactgtcagcggcaggacaacgtattcgatgtgttatctgaaagtactgatgaacggtgcggtgatttatgatggcgcggcgaacgaggcggtacaggtgttctcccgtattgttgacatgccagcgggtcggggaaacgtgatcctgacgttcacgcttacgtccacacggcattcggcagatattccgccgtatacgtttgccagcgatgtgcaggttatggtgattaagaaacaggcgctgggcatcagcgtggtctgagtgtgttacagaggttcgtccgggaacgggcgttttattataaaacagtgagaggtgaacgatgcgtaatgtgtgtattgccgttgctgtctttgccgcacttgcggtgacccggaatgaaattaatacgactcactatagggagataaggaggggctattaatggaaccttttaaatatatatgccattactggggaaaatcctcaaaaagcttgacgaaaggaaatgatattcatctgttaatttatcattgccttgatgttgctgctgttgcagattgctggtgggatcaatcagtcgtactgcaaaatactttttgccgaaatgaaatgctatcaaaacagagggtgaaggcctggctgttatttttcattgctcttcatgatattggaaagtttgatatacgattccaatataaatcagcagaaagttggctgaaattaaatcctgcaacgccatcacttaatggtccatcaacacaaatgtgccgtaaatttaatcatggtgcagccggtctgtattggtttaaccaggattcactttcagagcaatctctcggggattttttcagtttttttgatgccgctcctcatccttatgagtcctggtttccatgggtagaggccgttacaggacatcatggttttatattacattcccaggatcaagataagtcgcgttgggaaatgccagcttctctggcatcttatgctgcgcaagataaacaggctcgtgaggagtggatatctgtactggaagcattatttttaacgccagcggggttatctataaacgatataccacctgattgttcatcactgttagcaggtttttgctcgcttgctgactggttaggctcctggactacaacgaatacctttctgtttaatgaggatgcgccttccgacataaatgctctgagaacgtatttccaggaccgacagcaggatgcgagccgggtattggagttgagtggacttgtatcaaataagcgatgttatgaaggtgttcatgcactactggacaatggctatcaacccagacaattacaggtgttagttgatgctcttccagtagctcccgggctgacggtaatagaggcacctacaggctccggtaaaacggaaacagcgctggcctatgcttggaaacttattgatcaacaaattgcggatagtgttatttttgccctcccaacacaagctaccgcgaatgctatgcttacgagaatggaagcgagcgcgagccacttattttcatccccaaatcttattcttgctcatggcaattcacggtttaaccacctctttcaatcaataaaatcacgcgcgattactgaacaggggcaagaagaagcgtgggttcagtgttgtcagtggttgtcacaaagcaataagaaagtgtttcttgggcaaatcggcgtttgcacgattgatcaggtgttgatatcggtattgccagttaaacaccgctttatccgtggtttgggaattggtcgaagtgttttaattgttgatgaagttcatgcttacgacacctatatgaacggcttgctggaggcagtgctcaaggctcaggctgatgtgggagggagtgttattcttctttccgcaaccctaccaatgaaacaaaaacagaaacttctggatacttatggtctgcatacagatccagtggaaaataactccgcatatccactcattaactggcgaggtgtgaatggtgcgcaacgttttgatctgctagctcatccagaacaactcccgccccgcttttcgattcagccagaacctatttgtttagctgacatgttacctgaccttacgatgttagagcgaatgatcgcagcggcaaacgcgggtgcacaggtctgtcttatttgcaatttggttgacgttgcacaagtatgctaccaacggctaaaggagctaaataacacgcaagtagatatagatttgtttcatgcgcgctttacgctgaacgatcgtcgtgaaaaagagaatcgagttattagcaatttcggcaaaaatgggaagcgaaatgttggacggatacttgtcgcaacccaggtcgtggaacaatcactcgacgttgattttgattggttaattactcagcattgtcctgcagatttgcttttccaacgattgggccgtttacatcgccatcatcgcaaatatcgtcccgctggttttgagattcctgttgccaccattttgctgcctgatggcgagggttacggacgacatgagcatatttatagcaacgttagagtcatgtggcggacgcagcaacatattgaggagcttaatggagcatccttatttttccctgatgcttaccggcaatggctggatagcatttacgatgatgcggaaatggatgagccagaatgggtcggcaatggcatggataaatttgaaagcgccgagtgtgaaaaaaggttcaaggctcgcaaggtcctgcagtgggctgaagaatatagcttgcaggataacgatgaaaccattcttgcggtaacgagggatggggaaatgagcctgccattattgccttatgtacaaacgtcttcaggtaaacaactgctcgatggccaggtctacgaggacctaagtcatgaacagcagtatgaggcgcttgcacttaatcgcgtcaatgtacccttcacctggaaacgtagtttttctgaagtagtagatgaagatgggttactttggctggaagggaaacagaatctggatggatgggtctggcagggtaacagtattgttattacctatacaggggatgaagggatgaccagagtcatccctgcaaatcccaaataacttcgggaatgattgttatcaatgacgataataagaccaataacggtttatgtgtaggctggagctgcttcgaagttcctatactttctagagaataggaacttcggaataggaactaaggaggatattcagaaattaatacgactcactatagggagataaggagggagaacaaatgaatttgcttattgataactggatccctgtacgcccgcgaaacggggggaaagtccaaatcataaatctgcaatcgctatactgcagtagagatcagtggcgattaagtttgccccgtgacgatatggaactggccgctttagcactgctggtttgcattgggcaaattatcgccccggcaaaagatgacgttgaatttcgacatcgcataatgaatccgctcactgaagatgagtttcaacaactcatcgcgccgtggatagatatgttctaccttaatcacgcagaacatccctttatgcagaccaaaggtgtcaaagcaaatgatgtgactccaatggaaaaactgttggctggggtaagcggcgcgacgaattgtgcatttgtcaatcaaccggggcagggtgaagcattatgtggtggatgcactgcgattgcgttattcaaccaggcgaatcaggcaccaggttttggtggtggttttaaaagcggtttacgtggaggaacacctgtaacaacgttcgtacgtgggatcgatcttcgttcaacggtgttactcaatgtcctcacattacctcgtcttcaaaaacaatttcctaatgaatcacatacggaaaaccaacctacctggattaaacctatcaagtccaatgagtctatacctgcttcgtcaattgggtttgtccgtggtctattctggcaaccagcgcatattgaattatgcgatcccattgggattggtaaatgttcttgctgtggacaggaaagcaatttgcgttataccggttttcttaaggaaaaatttacctttacagttaatgggctatggccccatccgcattccccttgtctggtaacagtcaagaaaggggaggttgaggaaaaatttcttgctttcaccacctccgcaccatcatggacacaaatcagccgagttgtggtagataagattattcaaaatgaaaatggaaatcgcgtggcggcggttgtgaatcaattcagaaatattgcgccgcaaagtcctcttgaattgattatggggggatatcgtaataatcaagcatctattcttgaacggcgtcatgatgtgttgatgtttaatcaggggtggcaacaatacggcaatgtgataaacgaaatagtgactgttggtttgggatataaaacagccttacgcaaggcgttatatacctttgcagaagggtttaaaaataaagacttcaaaggggccggagtctctgttcatgagactgcagaaaggcatttctatcgacagagtgaattattaattcccgatgtactggcgaatgttaatttttcccaggctgatgaggtaatagctgatttacgagacaaacttcatcaattgtgtgaaatgctatttaatcaatctgtagctccctatgcacatcatcctaaattaataagcacattagcgcttgcccgcgccacgctatacaaacatttacgggagttaaaaccgcaaggagggccatcaaatggctgatgaaattgatgcaatggctttatatcgagcctggcaacaactggataatggatcatgtgcgcaaattagacgtgtttcagaacctgatgaattacgcgatatccctgcgttttataggctggtgcaaccttttggttgggaaaacccacgtcaccagcaggctcttttgcgcatggtgttttgcctgagcgcaggaaagaatgtcatccgacatcaggacaaaaaatcggagcaaacaacaggtatctcgttgggaagagctttagccaatagtggaagaattaacgagcgccgtatctttcaattaattcgggctgacagaacagccgatatggtccagttacgtcgattacttactcacgccgaacccgtacttgactggccattaatggccaggatgttgacctggtggggaaagcgcgaacgccagcaacttctggaagattttgtattgaccacaaacaaaaatgcgtaaggaaacctttctatgtctaactttatcaatattcatgttctgatctctcacagcccttcatgtctgaaccgcgacgatatgaacatgcagaaagacgctattttcggcggcaaaagacgagtaagaatttcaagtcaaagccttaaacgtgcgatgcgtaaaagtggttattacgcacaaaatattggtgaatccagtctcagaaccattcatcttgcacaattacgtgatgttcttcggcaaaaacttggtgaacgttttgaccaaaaaatcatcgataagacattagcgctgctctccggtaaatcagttgatgaagccgaaaagatttctgccgatgcggttactccctgggttgtgggagaaatagcctggttctgtgagcaggttgcaaaagcagaggctgataatctggatgataaaaagctgctcaaagttcttaaggaagatattgccgccatacgtgtgaatttacagcagggtgttgatattgcgcttagtggaagaatggcaaccagcggcatgatgactgagttgggaaaagttgatggtgcaatgtccattgcgcatgcgatcactactcatcaggttgattctgatattgactggttcaccgctgtagatgatttacaggaacaaggttctgcacatctgggaactcaggaattttcatcgggtgttttttatcgttatgccaacattaacctcgctcaacttcaggaaaatttaggtggtgcctccagggagcaggctctggaaattgcaacccatgttgttcatatgctggcaacagaggtccctggagcaaaacagcgtacttatgccgcttttaaccctgcggatatggtaatggttaatttctccgatatgccactttctatggcaaatgcttttgaaaaagcggttaaagcgaaagatggctttttgcaaccgtctatacaggcgtttaatcaatattgggatcgcgttgccaatggatatggtctgaacggagctgctgcgcaattcagcttatctgatgtagacccaattactgctcaagttaaacaaatgcctactttagaacagttaaaatcctgggttcgtaataatggcgaggcgtgaacatgagatcttatttgatcttgcggcttgctgggccaatgcaagcctgggggcagccgacctttgaaggaacgcgacctaccggaagatttccgacccgaagcgggttattagggctactcggggcttgtcttgggatccaacgtgatgatacttcttcattacaggcgttatcagagagtgtgcaatttgcagtgcgctgcgatgaactcattcttgacgatcgtcgtgtgtctgtaacggggttgcgtgattaccatacagtccttggagcgcgagaagattaccgtggtttgaaaagtcatgaaacgattcaaacatggcgcgaatatttatgtgatgcctcctttaccgtcgctctctggttaacaccccatgcaacgatggttatctcagaacttgaaaaagcagtattaaagcctcggtatacaccttacctggggcggagaagttgcccactaacacacccgctttttttggggacatgtcaggcatcggatcctcagaaggcgctattaaattatgagcccgttggcggcgatatatatagtgaggaatcagttacagggcatcatttaaaatttacggcgcgcgacgaaccgatgatcaccttgcctcgacaatttgcttcccgagaatggtatgtgattaaaggaggtatggatgtatctcagtaaagtcatcattgccagggcctggagcagggatctttaccaacttcaccagggattatggcatttatttccaaacagaccggatgctgctcgtgattttctttttcatgttgagaagcgaaacacaccagaaggctgtcatgttttattgcagtcagcgcaaatgcctgtttcaactgccgttgcgacagtcattaaaactaaacaggttgaatttcaacttcaggttggtgttccactctattttcggcttcgggcaaatccgatcaaaactattctcgacaatcaaaagcgcctggacagtaaagggaatattaaacgctgtcgggttccgttaataaaagaagcagaacaaatcgcgtggttgcaacgtaaattgggcaatgcggcgcgcgttgaagatgtgcatcccatatcggaacggccacagtatttttctggtgatggtaaaagtggaaagatccaaacggtttgctttgaaggtgtgctcaccatcaacgacgcgccagcgttaatagatcttgtacagcaaggtattgggccagctaaatcgatgggatgtggcttgctatctttggctccactgtgagggatgtgctgcaaggcgattaagttgggtaacgccagggttttcccagtcacgacgttgtaaaacgacggccagtgaattcaattaatacgactcactatagggcccgggggatccggaaaacaaagaattagctgatctttaataataaggaaatgttacattaaggttggtgggttgtttttatgggaaaaaatgctttaagaacaaatgtatacttttagagagttccccgcgccagcggggataaaccgctgagcaccgcattagccgctgcattgatgctgagttccccgcgccagcggggataaaccgcaggagatcaacctgccggtcgcgctggcggtgagttccccgcgccagcggggataaaccgcgatgtcggtgccgtcgatcccaacggtgatagagttccccgcgccagcggggataaaccgtgtgccgctgtatgcgcaaacggcggacgtacgagttccccgcgccagcggggataaaccgctgattgctcacgttggcggcccggctagcgtgagttccccgcgccagcggggataaaccgcaggcagtccagcctgaatgctcgctgcaccggagttccccgcgccagcggggataaaccggatcgtatgctatccattacaccagcgggacggagttccccgcgccagcggggataaaccgtctgcatcacgagtacctttcatagtacgaatgagttccccgcgccagcggggataaaccgcggagggcaagaaatagcttcacggtccatatgagttccccgcgccagcggggataaaccggtgatatcgcatgcaagctttgaatatcctccttagttcctattccgaagttcctattctctagaaagtataggaacttcggcgcgcctacctgtgacggaagatcacttcgcagaataaataaatcctggtgtccctgttgataccgggaagccctgggccaacttttggcgaaaatgagacgttgatcggcacgtaagaggttccaactttcaccataatgaaataagatcactaccgggcgtattttttgagttgtcgagattttcaggagctaaggaagctaaaatggagaaaaaaatcactggatataccaccgttgatatatcccaatggcatcgtaaagaacattttgaggcatttcagtcagttgctcaatgtacctataaccagaccgttcagctggatattacggcctttttaaagaccgtaaagaaaaataagcacaagttttatccggcctttattcacattcttgcccgcctgatgaatgctcatccggaattacgtatggcaatgaaagacggtgagctggtgatatgggatagtgttcacccttgttacaccgttttccatgagcaaactgaaacgttttcatcgctctggagtgaataccacgacgatttccggcagtttctacacatatattcgcaagatgtggcgtgttacggtgaaaacctggcctatttccctaaagggtttattgagaatatgtttttcgtctcagccaatccctgggtgagtttcaccagttttgatttaaacgtggccaatatggacaacttcttcgcccccgttttcaccatgggcaaatattatacgcaaggcgacaaggtgctgatgccgctggcgattcaggttcatcatgccgtttgtgatggcttccatgtcggcagatgcttaatgaatacaacagtactgcgatgagtggcagggcggggcgtaaggcgcgccatttaaatgaagttcctattccgaagttcctattctctagaaagtataggaacttcgaagcagctccagcctacacttgacatgaggttgccccgtgctttgcactggattgcgaggctttgtgcttctctggagtgcgacaggtttgatgacaaaaaattagcgcaagaagacaaaaatcaccttgcgctaatgctctgttacaggtcactaataccatctaagtagttgattcatagtgactgcatatgttgtgttttacagtattatgtagtctgttttttatgcaaaatctaatttaatatattgatatttatatcattttacgtttctcgttcagcttttttatactaagttggcattataaaaaagcattgcttatcaatttgttgcaacgaacaggtcactatcagtcaaaataaaatcattatttgatttcaattttgtcccactccctgcctctgtcatcacgatactgtgatgccatggtgtccgacttatgcccgagaagatgttgagcaaacttatcgcttatctgcttctcatagagtcttgcagacaaactgcgcaactcgtgaaaggtaggcggatccccttcgaaggaaagacctgatgcttttcgtgcgcgcataaaataccttgatactgtgccggatgaaagcggttcgcgacgagtagatgcaattatggtttctccgccaagaatctctttgcatttatcaagtgtttccttcattgatattccgagagcatcaatatgcaatgctgttgggatggcaatttttacgcctgttttgctttgctcgacataaagatatccatctacgatatcagaccacttcatttcgcataaatcaccaactcgttgcccggtaacaacagccagttccattgcaagtctgagccaacatggtgatgattctgctgcttgataaattttcaggtattcgtcagccgtaagtcttgatctccttacctctgattttgctgcgcgagtggcagcgacatggtttgttgttatatggccttcagctattgcctctcggaatgcatcgctcagtgttgatctgattaacttggctgacgccgccttgccctcgtctatgtatccattgagcattgccgcaatttcttttgtggtgatgtcttcaagtggagcatcaggcagacccctccttattgctttaattttgctcatgtaatttatgagtgtcttctgcttgattcctctgctggccaggattttttcgtagcgatcaagccatgaatgtaacgtaacggaattatcactgttgattctcgctgtcagaggcttgtgtttgtgtcctgaaaataactcaatgttggcctgtatagcttcagtgattgcgattcgcctgtctctgcctaatccaaactctttacccgtccttgggtccctgtagcagtaatatccattgtttcttatataaaggttagggggtaaatcccggcgctcatgacttcgccttcttcccatttctgatcctcttcaaaaggccacctgttactggtcgatttaagtcaacctttaccgctgattcgtggaacagatactctcttccatccttaaccggaggtgggaatatcctgcattcccgaacccatcgacgaactgtttcaaggcttcttggacgtcgctggcgtgcgttccactcctgaagtgtcaagtacatcgcaaagtctccgcaattacacgcaagaaaaaaccgccatcaggcggcttggtgttctttcagttcttcaattcgaatattggttacgtctgcatgtgctatctgcgcccatatcatccagtggtcgtagcagtcgttgatgttctccgcttcgataactctgttgaatggctctccattccattctcctgtgactcggaagtgcatttatcatctccataaaacaaaacccgccgtagcgagttcagataaaataaatccccgcgagtgcgaggattgttatgtaatattgggtttaatcatctatatgttttgtacagagagggcaagtatcgtttccaccgtactcgtgataataattttgcacggtatcagtcatttctcgcacattgcagaatggggatttgtcttcattagacttataaaccttcatggaatatttgtatgccgactctatatctataccttcatctacataaacaccttcgtgatgtctgcatggagacaagacaccggatctgcacaacattgataacgcccaatctttttgctcagactctaactcattgatactcatttataaactccttgcaatgtatgtcgtttcagctaaacggtatcagcaatgtttatgtaaagaaacagtaagataatactcaacccgatgtttgagtacggtcatcatctgacactacagactctggcatcgctgtgaagacgacgcgaaattcagcattttcacaagcgttatcttttacaaaaccgatctcactctcctttgatgcgaatgccagcgtcagacatcatatgcagatactcacctgcatcctgaacccattgacctccaaccccgtaatagcgatgcgtaatgatgtcgatagttactaacgggtcttgttcgattaactgccgcagaaactcttccaggtcaccagtgcagtgcttgataacaggagtcttcccaggatggcgaacaacaagaaactggtttccgtcttcacggacttcgttgctttccagtttagcaatacgcttactcccatccgagataacaccttcgtaatactcacgctgctcgttgagttttgattttgctgtttcaagctcaacacgcagtttccctactgttagcgcaatatcctcgttctcctggtcgcggcgtttgatgtattgctggtttctttcccgttcatccagcagttccagcacaatcgatggtgttaccaattcatggaaaaggtctgcgtcaaatccccagtcgtcatgcattgcctgctctgccgcttcacgcagtgcctgagagttaatttcgctcacttcgaacctctctgtttactgataagttccagatcctcctggcaacttgcacaagtccgacaaccctgaacgaccaggcgtcttcgttcatctatcggatcgccacactcacaacaatgagtggcagatatagcctggtggttcaggcggcgcatttttattgctgtgttgcgctgtaattcttctatttctgatgctgaatcaatgatgtctgccatctttcattaatccctgaactgttggttaatacgcttgagggtgaatgcgaataataaaaaaggagcctgtagctccctgatgattttgcttttcatgttcatcgttccttaaagacgccgtttaacatgccgattgccaggcttaaatgagtcggtgtgaatcccatcagcgttaccgtttcgcggtgcttcttcagtacgctacggcaaatgtcatcgacgtttttatccggaaactgctgtctggctttttttgatttcagaattagcctgacgggcaatgctgcgaagggcgttttcctgctgaggtgtcattgaacaagtcccatgtcggcaagcataagcacacagaatatgaagcccgctgccagaaaaatgcattccgtggttgtcatacctggtttctctcatctgcttctgctttcgccaccatcatttccagcttttgtgaaagggatgcggctaacgtatgaaattcttcgtctgtttctactggtattggcacaaacctgattccaatttgagcaaggctatgtgccatctcgatactcgttcttaactcaacagaagatgctttgtgcatacagcccctcgtttattatttatctcctcagccagccgctgtgctttcagtggatttcggataacagaaaggccgggaaatacccagcctcgctttgtaacggagtagacgaaagtgattgcgcctacccggatattatcgtgaggatgcgtcatcgccattgctccccaaatacaaaaccaatttcagccagtgcctcgtccattttttcgatgaactccggcacgatctcgtcaaaactcgccatgtacttttcatcccgctcaatcacgacataatgcaggccttcacgcttcatacgcgggtcatagttggcaaagtaccaggcattttttcgcgtcacccacatgctgtactgcacctgggccatgtaagctgactttatggcctcgaaaccaccgagccggaacttcatgaaatcccgggaggtaaacgggcatttcagttcaaggccgttgccgtcactgcataaaccatcgggagagcaggcggtacgcatactttcgtcgcgatagatgatcggggattcagtaacattcacgccggaagtgaattcaaacagggttctggcgtcgttctcgtactgttttccccaggccagtgctttagcgttaacttccggagccacaccggtgcaaacctcagcaagcagggtgtggaagtaggacattttcatgtcaggccacttctttccggagcggggttttgctatcacgttgtgaacttctgaagcggtgatgacgccgagccgtaatttgtgccacgcatcatccccctgttcgacagctctcacatcgatcccggtacgctgcaggataatgtccggtgtcatgctgccaccttctgctctgcggctttctgtttcaggaatccaagagcttttactgcttcggcctgtgtcagttctgacgatgcacgaatgtcgcggcgaaatatctgggaacagagcggcaataagtcgtcatcccatgttttatccagggcgatcagcagagtgttaatctcctgcatggtttcatcgttaaccggagtgatgtcgcgttccggctgacgttctgcagtgtatgcagtattttcgacaatgcgctcggcttcatccttgtcatagataccagcaaatccgaaggccagacgggcacactgaatcatggctttatgacgtaacatccgtttgggatgcgactgccacggccccgtgatttctctgccttcgcgagttttgaatggttcgcggcggcattcatccatccattcggtaacgcagatcggatgattacggtccttgcggtaaatccggcatgtacaggattcattgtcctgctcaaagtccatgccatcaaactgctggttttcattgatgatgcgggaccagccatcaacgcccaccaccggaacgatgccattctgcttatcaggaaaggcgtaaatttctttcgtccacggattaaggccgtactggttggcaacgatcagtaatgcgatgaactgcgcatcgctggcatcacctttaaatgccgtctggcgaagagtggtgatcagttcctgtgggtcgacagaatccatgccgacacgttcagccagcttcccagccagcgttgcgagtgcagtactcattcgttttatacctctgaatcaatatcaacctggtggtgagcaatggtttcaaccatgtaccggatgtgttctgccatgcgctcctgaaactcaacatcgtcatcaaacgcacgggtaatggattttttgctggccccgtggcgttgcaaatgatcgatgcatagcgattcaaacaggtgctggggcaggcctttttccatgtcgtctgccagttctgcctctttctcttcacgggcgagctgctggtagtgacgcgcccagctctgagcctcaagacgatcctgaatgtaataagcgttcatggctgaactcctgaaatagctgtgaaaatatcgcccgcgaaatgccgggctgattaggaaaacaggaaagggggttagtgaatgcttttgcttgatctcagtttcagtattaatatccattttttataagcgtcgacggcttcacgaaacatcttttcatcgccaataaaagtggcgatagtgaatttagtctggatagccataagtgtttgatccattctttgggactcctggctgattaagtatgtcgataaggcgtttccatccgtcacgtaatttacgggtgattcgttcaagtaaagattcggaagggcagccagcaacaggccaccctgcaatggcatattgcatggtgtgctccttatttatacataacgaaaaacgcctcgagtgaagcgttattggtatgcggtaaaaccgcactcaggcggccttgatagtcatatcatctgaatcaaatattcctgatgtatcgatatcggtaattcttattccttcgctaccatccattggaggccatccttcctgaccatttccatcattccagtcgaactcacacacaacaccatatgcatttaagtcgcttgaaattgctataagcagagcatgttgcgccagcatgattaatacagcatttaatacagagccgtgtttattgagtcggtattcagagtctgaccagaaattattaatctggtgaagtttttcctctgtcattacgtcatggtcgatttcaatttctattgatgctttccagtcgtaatcaatgatgtattttttgatgtttgacatctgttcatatcctcacagataaaaaatcgccctcacactggagggcaaagaagatttccaataatcagaacaagtcggctcctgtttagttacgagcgacattgctccgtgtattcactcgttggaatgaatacacagtgcagtgtttattctgttatttatgccaaaaataaaggccactatcaggcagctttgttgttctgtttaccaagttctctggcaatcattgccgtcgttcgtattgcccatttatcgacatatttcccatcttccattacaggaaacatttcttcaggcttaaccatgcattccgattgcagcttgcatccattgcatcgcttgaattgtccacaccattgatttttatcaatagtcgtagtcatacggatagtcctggtattgttccatcacatcctgaggatgctcttcgaactcttcaaattcttcttccatatatcaccttaaatagtggattgcggtagtaaagattgtgcctgtcttttaaccacatcaggctcggtggttctcgtgtacccctacagcgagaaatcggataaactattacaacccctacagtttgatgagtatagaaatggatccactcgttattctcggacgagtgttcagtaatgaacctctggagagaaccatgtatatgatcgttatctgggttggacttctgcttttaagcccagataactggcctgaatatgttaatgagagaatcggtattcctcatgtgtggcatgttttcgtctttgctcttgcattttcgctagcaattaatgtgcatcgattatcagctattgccagcgccagatataagcgatttaagctaagaaaacgcattaagatgcaaaacgataaagtgcgatcagtaattcaaaaccttacagaagagcaatctatggttttgtgcgcagcccttaatgaaggcaggaagtatgtggttacatcaaaacaattcccatacattagtgagttgattgagcttggtgtgttgaacaaaactttttcccgatggaatggaaagcatatattattccctattgaggatatttactggactgaattagttgccagctatgatccatataatattgagataaagccaaggccaatatctaagtaactagataagaggaatcgattttcccttaattttctggcgtccactgcatgttatgccgcgttcgccaggcttgctgtaccatgtgcgctgattcttgcgctcaatacgttgcaggttgctttcaatctgtttgtggtattcagccagcactgtaaggtctatcggatttagtgcgctttctactcgtgatttcggtttgcgattcagcgagagaatagggcggttaactggttttgcgcttaccccaaccaacaggggatttgctgctttccattgagcctgtttctctgcgcgacgttcgcggcggcgtgtttgtgcatccatctggattctcctgtcagttagctttggtggtgtgtggcagttgtagtcctgaacgaaaaccccccgcgattggcacattggcagctaatccggaatcgcacttacggccaatgcttcgtttcgtatcacacaccccaaagccttctgctttgaatgctgcccttcttcagggcttaatttttaagagcgtcaccttcatggtggtcagtgcgtcctgctgatgtgctcagtatcaccgccagtggtatttatgtcaacaccgccagagataatttatcaccgcagatggttatctgtatgttttttatatgaatttattttttgcaggggggcattgtttggtaggtgagagatctgaattgctatgtttagtgagttgtatctatttatttttcaataaatacaattggttatgtgttttgggggcgatcgtgaggcaaagaaaacccggcgctgaggccgggttattcttgttctctggtcaaattatatagttggaaaacaaggatgcatatatgaatgaacgatgcagaggcaatgccgatggcgatagtgggtatcatgtagccgcttatgctggaaagaagcaataacccgcagaaaaacaaagctccaagctcaacaaaactaagggcatagacaataactaccgatgtcatatacccatactctctaatcttggccagtcggcgcgttctgcttccgattagaaacgtcaaggcagcaatcaggattgcaatcatggttcctgcatatgatgacaatgtcgccccaagaccatctctatgagctgaaaaagaaacaccaggaatgtagtggcggaaaaggagatagcaaatgcttacgataacgtaaggaattattactatgtaaacaccaggcatgattctgttccgcataattactcctgataattaatccttaactttgcccacctgccttttaaaacattccagtatatcacttttcattcttgcgtagcaatatgccatctcttcagctatctcagcattggtgaccttgttcagaggcgctgagagatggcctttttctgatagataatgttctgttaaaatatctccggcctcatcttttgcccgcaggctaatgtctgaaaattgaggtgacgggttaaaaataatatccttggcaaccttttttatatcccttttaaattttggcttaatgactatatccaatgagtcaaaaagctccccttcaatatctgttgcccctaagacctttaatatatcgccaaatacaggtagcttggcttctaccttcaccgttgttcggccgatgaaatgcatatgcataacatcgtctttggtggttcccctcatcagtggctctatctgaacgcgctctccactgcttaatgacattcctttcccgattaaaaaatctgtcagatcggatgtggtcggcccgaaaacagttctggcaaaaccaatggtgtcgccttcaacaaacaaaaaagatgggaatcccaatgattcgtcatctgcgaggctgttcttaatatcttcaactgaagctttagagcgatttatcttctgaaccagactcttgtcatttgttttggtaaagagaaaagtttttccatcgattttatgaatatacaaataattggagccaacctgcaggtgatgattatcagccagcagagaattaaggaaaacagacaggtttattgagcgcttatctttccctttatttttgctgcggtaagtcgcataaaaaccattcttcataattcaatccatttactatgttatgttctgaggggagtgaaaattcccctaattcgatgaagattcttgctcaattgttatcagctatgcgccgaccagaacaccttgccgatcagccaaacgtctcttcaggccactgactagcgataactttccccacaacggaacaactctcattgcatgggatcattgggtactgtgggtttagtggttgtaaaaacacctgaccgctatccctgatcagtttcttgaaggtaaactcatcacccccaagtctggctatgcagaaatcacctggctcaacagcctgctcagggtcaacgagaattaacattccgtcaggaaagcttggcttggagcctgttggtgcggtcatggaattaccttcaacctcaagccagaatgcagaatcactggcttttttggttgtgcttacccatctctccgcatcacctttggtaaaggttctaagctcaggtgagaacatccctgcctgaacatgagaaaaaacagggtactcatactcacttctaagtgacggctgcatactaaccgcttcatacatctcgtagatttctctggcgattgaagggctaaattcttcaacgctaactttgagaatttttgcaagcaatgcggcgttataagcatttaatgcattgatgccattaaataaagcaccaacgcctgactgccccatccccatcttgtctgcgacagattcctgggataagccaagttcatttttctttttttcataaattgctttaaggcgacgtgcgtcctcaagctgctcttgtgttaatggtttcttttttgtgctcatacgttaaatctatcaccgcaagggataaatatctaacaccgtgcgtgttgactattttacctctggcggtgataatggttgcatgtactaaggaggttgtatggaacaacgcataaccctgaaagattatgcaatgcgctttgggcaaaccaagacagctaaagatctcggcgtatatcaaagcgcgatcaacaaggccattcatgcaggccgaaagatttttttaactataaacgctgatggaagcgtttatgcggaagaggtaaagcccttcccgagtaacaaaaaaacaacagcataaataaccccgctcttacacattccagccctgaaaaagggcatcaaattaaaccacacctatggtgtatgcatttatttgcatacattcaatcaattgttatctaaggaaatacttacatatggttcgtgcaaacaaacgcaacgaggctctacgaatcgagagtgcgttgcttaacaaaatcgcaatgcttggaactgagaagacagcggaagctgtgggcgttgataagtcgcagatcagcaggtggaagagggactggattccaaagttctcaatgctgcttgctgttcttgaatggggggtcgttgacgacgacatggctcgattggcgcgacaagttgctgcgattctcaccaataaaaaacgcccggcggcaaccgagcgttctgaacaaatccagatggagttctgaggtcattactggatctatcaacaggagtcattatgacaaatacagcaaaaatactcaacttcggcagaggtaactttgccggacaggagcgtaatgtggcagatctcgatgatggttacgccagactatcaaatatgctgcttgaggcttattcgggcgcagatctgaccaagcgacagtttaaagtgctgcttgccattctgcgtaaaacctatgggtggaataaaccaatggacagaatcaccgattctcaacttagcgagattacaaagttacctgtcaaacggtgcaatgaagccaagttagaactcgtcagaatgaatattatcaagcagcaaggcggcatgtttggaccaaataaaaacatctcagaatggtgcatccctcaaaacgagggaaaatcccctaaaacgagggataaaacatccctcaaattgggggattgctatccctcaaaacagggggacacaaaagacactattacaaaagaaaaaagaaaagattattcgtcagagaattctggcgaatcctctgaccagccagaaaacgacctttctgtggtgaaaccggatgctgcaattcagagcggcagcaagtgggggacagcagaagacctgaccgccgcagagtggatgtttgacatggtgaagactatcgcaccatcagccagaaaaccgaattttgctgggtgggctaacgatatccgcctgatgcgtgaacgtgacggacgtaaccaccgcgacatgtgtgtgctgttccgctgggcatgccaggacaacttctggtccggtaacgtgctgagcccggccaaactccgcgataagtggacccaactcgaaatcaaccgtaacaagcaacaggcaggcgtgacagccagcaaaccaaaactcgacctgacaaacacagactggatttacggggtggatctatgaaaaacatcgccgcacagatggttaactttgaccgtgagcagatgcgtcggatcgccaacaacatgccggaacagtacgacgaaaagccgcaggtacagcaggtagcgcagatcatcaacggtgtgttcagccagttactggcaactttcccggcgagcctggctaaccgtgaccagaacgaagtgaacgaaatccgtcgccagtgggttctggcttttcgggaaaacgggatcaccacgatggaacaggttaacgcaggaatgcgcgtagcccgtcggcagaatcgaccatttctgccatcacccgggcagtttgttgcatggtgccgggaagaagcatccgttaccgccggactgccaaacgtcagcgagctggttgatatggtttacgagtattgccggaagcgaggcctgtatccggatgcggagtcttatccgtggaaatcaaacgcgcactactggctggttaccaacctgtatcagaacatgcgggccaatgcgcttactgatgcggaattacgccgtaaggccgcagatgagcttgtccatatgactgcgagaattaaccgtggtgaggcgatccctgaaccagtaaaacaacttcctgtcatgggcggtagacctctaaatcgtgcacaggctctggcgaagatcgcagaaatcaaagctaagttcggactgaaaggagcaagtgtatgacgggcaaagaggcaattattcattacctggggacgcataatagcttctgtgcgccggacgttgccgcgctaacaggcgcaacagtaaccagcataaatcaggccgcggctaaaatggcacgggcaggtcttctggttatcgaaggtaaggtctggcgaacggtgtattaccggtttgctaccagggaagaacgggaaggaaagatgagcacgaacctggtttttaaggagtgtcgccagagtgccgcgatgaaacgggtattggcggtatatggagttaaaagatgaccatctacattactgagctaataacaggcctgctggtaatcgcaggcctttttatttgggggagagggaagtcatgaaaaaactaacctttgaaattcgatctccagcacatcagcaaaacgctattcacgcagtacagcaaatccttccagacccaaccaaaccaatcgtagtaaccattcaggaacgcaaccgcagcttagaccaaaacaggaagctatgggcctgcttaggtgacgtctctcgtcaggttgaatggcatggtcgctggctggatgcagaaagctggaagtgtgtgtttaccgcagcattaaagcagcaggatgttgttcctaaccttgccgggaatggctttgtggtaataggccagtcaaccagcaggatgcgtgtaggcgaatttgcggagctattagagcttatacaggcattcggtacagagcgtggcgttaagtggtcagacgaagcgagactggctctggagtggaaagcgagatggggagacagggctgcatgataaatgtcgttagtttctccggtggcaggacgtcagcatatttgctctggctaatggagcaaaagcgacgggcaggtaaagacgtgcattacgttttcatggatacaggttgtgaacatccaatgacatatcggtttgtcagggaagttgtgaagttctgggatataccgctcaccgtattgcaggttgatatcaacccggagcttggacagccaaatggttatacggtatgggaaccaaaggatattcagacgcgaatgcctgttctgaagccatttatcgatatggtaaagaaatatggcactccatacgtcggcggcgcgttctgcactgacagattaaaactcgttcccttcaccaaatactgtgatgaccatttcgggcgagggaattacaccacgtggattggcatcagagctgatgaaccgaagcggctaaagccaaagcctggaatcagatatcttgctgaactgtcagactttgagaaggaagatatcctcgcatggtggaagcaacaaccattcgatttgcaaataccggaacatctcggtaactgcatattctgcattaaaaaatcaacgcaaaaaatcggacttgcctgcaaagatgaggagggattgcagcgtgtttttaatgaggtcatcacgggatcccatgtgcgtgacggacatcgggaaacgccaaaggagattatgtaccgaggaagaatgtcgctggacggtatcgcgaaaatgtattcagaaaatgattatcaagccctgtatcaggacatggtacgagctaaaagattcgataccggctcttgttctgagtcatgcgaaatatttggagggcagcttgatttcgacttcgggagggaagctgcatgatgcgatgttatcggtgcggtgaatgcaaagaagataaccgcttccgaccaaatcaaccttactggaatcgatggtgtctccggtgtgaaagaacaccaacaggggtgttaccactaccgcaggaaaaggaggacgtgtggcgagacagcgacgaagtatcaccgacataatctgcgaaaactgcaaataccttccaacgaaacgcaccagaaataaacccaagccaatcccaaaagaatctgacgtaaaaaccttcaactacacggctcacctgtgggatatccggtggctaagacgtcgtgcgaggaaaacaaggtgattgaccaaaatcgaagttacgaacaagaaagcgtcgagcgagctttaacgtgcgctaactgcggtcagaagctgcatgtgctggaagttcacgtgtgtgagcactgctgcgcagaactgatgagcgatccgaatagctcgatgcacgaggaagaagatgatggctaaaccagcgcgaagacgatgtaaaaacgatgaatgccgggaatggtttcaccctgcattcgctaatcagtggtggtgctctccagagtgtggaaccaagatagcactcgaacgacgaagtaaagaacgcgaaaaagcggaaaaagcagcagagaagaaacgacgacgagaggagcagaaacagaaagataaacttaagattcgaaaactcgccttaaagccccgcagttactggattaaacaagcccaacaagccgtaaacgccttcatcagagaaagagaccgcgacttaccatgtatctcgtgcggaacgctcacgtctgctcagtgggatgccggacattaccggacaactgctgcggcacctcaactccgatttaatgaacgcaatattcacaagcaatgcgtggtgtgcaaccagcacaaaagcggaaatctcgttccgtatcgcgtcgaactgattagccgcatcgggcaggaagcagtagacgaaatcgaatcaaaccataaccgccatcgctggactatcgaagagtgcaaggcgatcaaggcagagtaccaacagaaactcaaagacctgcgaaatagcagaagtgaggccgcatgacgttctcagtaaaaaccattccagacatgctcgttgaagcatacggaaatcagacagaagtagcacgcagactgaaatgtagtcgcggtacggtcagaaaatacgttgatgataaagacgggaaaatgcacgccatcgtcaacgacgttctcatggttcatcgcggatggagtgaaagagatgcgctattacgaaaaaattgatggcagcaaataccgaaatatttgggtagttggcgatctgcacggatgctacacgaacctgatgaacaaactggatacgattggattcgacaacaaaaaagacctgcttatctcggtgggcgatttggttgatcgtggtgcagagaacgttgaatgcctggaattaatcacattcccctggttcagagctgtacgtggaaaccatgagcaaatgatgattgatggcttatcagagcgtggaaacgttaatcactggctgcttaatggcggtggctggttctttaatctcgattacgacaaagaaattctggctaaagctcttgcccataaagcagatgaacttccgttaatcatcgaactggtgagcaaagataaaaaatatgttatctgccacgccgattatccctttgacgaatacgagtttggaaagccagttgatcatcagcaggtaatctggaaccgcgaacgaatcagcaactcacaaaacgggatcgtgaaagaaatcaaaggcgcggacacgttcatctttggtcatacgccagcagtgaaaccactcaagtttgccaaccaaatgtatatcgataccggcgcagtgttctgcggaaacctaacattgattcaggtacagggagaaggcgcatgagactcgaaagcgtagctaaatttcattcgccaaaaagcccgatgatgagcgactcaccacgggccacggcttctgactctctttccggtactgatgtgatggctgctatggggatggcgcaatcacaagccggattcggtatggctgcattctgcggtaagcacgaactcagccagaacgacaaacaaaaggctatcaactatctgatgcaatttgcacacaaggtatcggggaaataccgtggtgtggcaaagcttgaaggaaatactaaggcaaaggtactgcaagtgctcgcaacattcgcttatgcggattattgccgtagtgccgcgacgccgggggcaagatgcagagattgccatggtacaggccgtgcggttgatattgccaaaacagagctgtgggggagagttgtcgagaaagagtgcggaagatgcaaaggcgtcggctattcaaggatgccagcaagcgcagcatatcgcgctgtgacgatgctaatcccaaaccttacccaacccacctggtcacgcactgttaagccgctgtatgacgctctggtggtgcaatgccacaaagaagagtcaatcgcagacaacattttgaatgcggtcacacgttagcagcatgattgccacggatggcaacatattaacggcatgatattgacttattgaataaaattgggtaaatttgactcaacgatgggttaattcgctcgttgtggtagtgagatgaaaagaggcggcgcttactaccgattccgcctagttggtcacttcgacgtatcgtctggaactccaaccatcgcaggcagagaggtctgcaaaatgcaatcccgaaacagttcgcaggtaatagttagagcctgcataacggtttcgggattttttatatctgcacaacaggtaagagcattgagtcgataatcgtgaagagtcggcgagcctggttagccagtgctctttccgttgtgctgaattaagcgaataccggaagcagaaccggatcaccaaatgcgtacaggcgtcatcgccgcccagcaacagcacaacccaaactgagccgtagccactgtctgtcctgaattcattagtaatagttacgctgcggccttttacacatgaccttcgtgaaagcgggtggcaggaggtcgcgctaacaacctcctgccgttttgcccgtgcatatcggtcacgaacaaatctgattactaaacacagtagcctggatttgttctatcagtaatcgaccttattcctaattaaatagagcaaatccccttattgggggtaagacatgaagatgccagaaaaacatgacctgttggccgccattctcgcggcaaaggaacaaggcatcggggcaatccttgcgtttgcaatggcgtaccttcgcggcagatataatggcggtgcgtttacaaaaacagtaatcgacgcaacgatgtgcgccattatcgcctggttcattcgtgaccttctcgacttcgccggactaagtagcaatctcgcttatataacgagcgtgtttatcggctacatcggtactgactcgattggttcgcttatcaaacgcttcgctgctaaaaaagccggagtagaagatggtagaaatcaataatcaacgtaaggcgttcctcgatatgctggcgtggtcggagggaactgataacggacgtcagaaaaccagaaatcatggttatgacgtcattgtaggcggagagctatttactgattactccgatcaccctcgcaaacttgtcacgctaaacccaaaactcaaatcaacaggcgccggacgctaccagcttctttcccgttggtgggatgcctaccgcaagcagcttggcctgaaagacttctctccgaaaagtcaggacgctgtggcattgcagcagattaaggagcgtggcgctttacctatgattgatcgtggtgatatccgtcaggcaatcgaccgttgcagcaatatctgggcttcactgccgggcgctggttatggtcagttcgagcataaggctgacagcctgattgcaaaattcaaagaagcgggcggaacggtcagagagattgatgtatgagcagagtcaccgcgattatctccgctctggttatctgcatcatcgtctgcctgtcatgggctgttaatcattaccgtgataacgccattacctacaaagcccagcgcgacaaaaatgccagagaactgaagctggcgaacgcggcaattactgacatgcagatgcgtcagcgtgatgttgctgcgctcgatgcaaaatacacgaaggagttagctgatgctaaagctgaaaatgatgctctgcgtgatgatgttgccgctggtcgtcgtcggttgcacatcaaagcagtctgtcagtcagtgcgtgaagccaccaccgcctccggcgtggataatgcagcctccccccgactggcagacaccgctgaacgggattatttcaccctcagagagaggctgatcactatgcaaaaacaactggaaggaacccagaagtatattaatgagcagtgcagatagagttgcccatcgacctgcaggggggggggggcgctgaggtctgcctcgtgaagaaggtgttgctgactcataccaggcctgaatcgccccatcatccagccagaaagtgagggagccacggttgatgagagctttgttgtaggtggaccagttggtgattttgaacttttgctttgccacggaacggtctgcgttgtcgggaagatgcgtgatctgatccttcaactcagcaaaagttcgatttattcaacaaagccgccgtcccgtcaagtcagcgtaatgctctgccagtgttacaaccaattaaccaattctgattagaaaaactcatcgagcatcaaatgaaactgcaatttattcatatcaggattatcaataccatatttttgaaaaagccgtttctgtaatgaaggagaaaactcaccgaggcagttccataggatggcaagatcctggtatcggtctgcgattccgactcgtccaacatcaatacaacctattaatttcccctcgtcaaaaataaggttatcaagtgagaaatcaccatgagtgacgactgaatccggtgagaatggcaaaagcttatgcatttctttccagacttgttcaacaggccagccattacgctcgtcatcaaaatcactcgcatcaaccaaaccgttattcattcgtgattgcgcctgagcgagacgaaatacgcgatcgctgttaaaaggacaattacaaacaggaatcgaatgcaaccggcgcaggaacactgccagcgcatcaacaatattttcacctgaatcaggatattcttctaatacctggaatgctgttttcccggggatcgcagtggtgagtaaccatgcatcatcaggagtacggataaaatgcttgatggtcggaagaggcataaattccgtcagccagtttagtctgaccatctcatctgtaacatcattggcaacgctacctttgccatgtttcagaaacaactctggcgcatcgggcttcccatacaatcgatagattgtcgcacctgattgcccgacattatcgcgagcccatttatacccatataaatcagcatccatgttggaatttaatcgcggcctcgagcaagacgtttcccgttgaatatggctcataacaccccttgtattactgtttatgtaagcagacagttttattgttcatgatgatatatttttatcttgtgcaatgtaacatcagagattttgagacacaacgtggctttcccccccccccctgcaggtcgttgacatgaggttgccccgtattcagtgtcgctgatttgtattgtctgaagttgtttttacgttaagttgatgcagatcaattaatacgatacctgcgtcataattgattatttgacgtggtttgatggcctccacgcacgttgtgatatgtagatgataatcattatcactttacgggtcctttccggtgatccgacaggttacg

SEQ ID NO: 60 - DNA, 1509 bp, Escherichia coli
atgaatttgcttattgataactggatccctgtacgcccgcgaaacggggggaaagtccaaatcataaatctgcaatcgctatactgcagtagagatcagtggcgattaagtttgccccgtgacgatatggaactggccgctttagcactgctggtttgcattgggcaaattatcgccccggcaaaagatgacgttgaatttcgacatcgcataatgaatccgctcactgaagatgagtttcaacaactcatcgcgccgtggatagatatgttctaccttaatcacgcagaacatccctttatgcagaccaaaggtgtcaaagcaaatgatgtgactccaatggaaaaactgttggctggggtaagcggcgcgacgaattgtgcatttgtcaatcaaccggggcagggtgaagcattatgtggtggatgcactgcgattgcgttattcaaccaggcgaatcaggcaccaggttttggtggtggttttaaaagcggtttacgtggaggaacacctgtaacaacgttcgtacgtgggatcgatcttcgttcaacggtgttactcaatgtcctcacattacctcgtcttcaaaaacaatttcctaatgaatcacatacggaaaaccaacctacctggattaaacctatcaagtccaatgagtctatacctgcttcgtcaattgggtttgtccgtggtctattctggcaaccagcgcatattgaattatgcgatcccattgggattggtaaatgttcttgctgtggacaggaaagcaatttgcgttataccggttttcttaaggaaaaatttacctttacagttaatgggctatggccccatccgcattccccttgtctggtaacagtcaagaaaggggaggttgaggaaaaatttcttgctttcaccacctccgcaccatcatggacacaaatcagccgagttgtggtagataagattattcaaaatgaaaatggaaatcgcgtggcggcggttgtgaatcaattcagaaatattgcgccgcaaagtcctcttgaattgattatggggggatatcgtaataatcaagcatctattcttgaacggcgtcatgatgtgttgatgtttaatcaggggtggcaacaatacggcaatgtgataaacgaaatagtgactgttggtttgggatataaaacagccttacgcaaggcgttatatacctttgcagaagggtttaaaaataaagacttcaaaggggccggagtctctgttcatgagactgcagaaaggcatttctatcgacagagtgaattattaattcccgatgtactggcgaatgttaatttttcccaggctgatgaggtaatagctgatttacgagacaaacttcatcaattgtgtgaaatgctatttaatcaatctgtagctccctatgcacatcatcctaaattaataagcacattagcgcttgcccgcgccacgctatacaaacatttacgggagttaaaaccgcaaggagggccatcaaatggctga

SEQ ID NO: 61 - DNA, 483 bp, Escherichia coli
atggctgatgaaattgatgcaatggctttatatcgagcctggcaacaactggataatggatcatgtgcgcaaattagacgtgtttcagaacctgatgaattacgcgatatccctgcgttttataggctggtgcaaccttttggttgggaaaacccacgtcaccagcaggctcttttgcgcatggtgttttgcctgagcgcaggaaagaatgtcatccgacatcaggacaaaaaatcggagcaaacaacaggtatctcgttgggaagagctttagccaatagtggaagaattaacgagcgccgtatctttcaattaattcgggctgacagaacagccgatatggtccagttacgtcgattacttactcacgccgaacccgtacttgactggccattaatggccaggatgttgacctggtggggaaagcgcgaacgccagcaacttctggaagattttgtattgaccacaaacaaaaatgcgtaa

SEQ ID NO: 62 - DNA, 1092 bp, Escherichia coli
atgtctaactttatcaatattcatgttctgatctctcacagcccttcatgtctgaaccgcgacgatatgaacatgcagaaagacgctattttcggcggcaaaagacgagtaagaatttcaagtcaaagccttaaacgtgcgatgcgtaaaagtggttattacgcacaaaatattggtgaatccagtctcagaaccattcatcttgcacaattacgtgatgttcttcggcaaaaacttggtgaacgttttgaccaaaaaatcatcgataagacattagcgctgctctccggtaaatcagttgatgaagccgaaaagatttctgccgatgcggttactccctgggttgtgggagaaatagcctggttctgtgagcaggttgcaaaagcagaggctgataatctggatgataaaaagctgctcaaagttcttaaggaagatattgccgccatacgtgtgaatttacagcagggtgttgatattgcgcttagtggaagaatggcaaccagcggcatgatgactgagttgggaaaagttgatggtgcaatgtccattgcgcatgcgatcactactcatcaggttgattctgatattgactggttcaccgctgtagatgatttacaggaacaaggttctgcacatctgggaactcaggaattttcatcgggtgttttttatcgttatgccaacattaacctcgctcaacttcaggaaaatttaggtggtgcctccagggagcaggctctggaaattgcaacccatgttgttcatatgctggcaacagaggtccctggagcaaaacagcgtacttatgccgcttttaaccctgcggatatggtaatggttaatttctccgatatgccactttctatggcaaatgcttttgaaaaagcggttaaagcgaaagatggctttttgcaaccgtctatacaggcgtttaatcaatattgggatcgcgttgccaatggatatggtctgaacggagctgctgcgcaattcagcttatctgatgtagacccaattactgctcaagttaaacaaatgcctactttagaacagttaaaatcctgggttcgtaataatggcgaggcgtga

SEQ ID NO: 63 - DNA, 675 bp, Escherichia coli
atgagatcttatttgatcttgcggcttgctgggccaatgcaagcctgggggcagccgacctttgaaggaacgcgacctaccggaagatttccgacccgaagcgggttattagggctactcggggcttgtcttgggatccaacgtgatgatacttcttcattacaggcgttatcagagagtgtgcaatttgcagtgcgctgcgatgaactcattcttgacgatcgtcgtgtgtctgtaacggggttgcgtgattaccatacagtccttggagcgcgagaagattaccgtggtttgaaaagtcatgaaacgattcaaacatggcgcgaatatttatgtgatgcctcctttaccgtcgctctctggttaacaccccatgcaacgatggttatctcagaacttgaaaaagcagtattaaagcctcggtatacaccttacctggggcggagaagttgcccactaacacacccgctttttttggggacatgtcaggcatcggatcctcagaaggcgctattaaattatgagcccgttggcggcgatatatatagtgaggaatcagttacagggcatcatttaaaatttacggcgcgcgacgaaccgatgatcaccttgcctcgacaatttgcttcccgagaatggtatgtgattaaaggaggtatggatgtatctcagtaa

SEQ ID NO: 64 - DNA, 600 bp, Escherichia coli
atgtatctcagtaaagtcatcattgccagggcctggagcagggatctttaccaacttcaccagggattatggcatttatttccaaacagaccggatgctgctcgtgattttctttttcatgttgagaagcgaaacacaccagaaggctgtcatgttttattgcagtcagcgcaaatgcctgtttcaactgccgttgcgacagtcattaaaactaaacaggttgaatttcaacttcaggttggtgttccactctattttcggcttcgggcaaatccgatcaaaactattctcgacaatcaaaagcgcctggacagtaaagggaatattaaacgctgtcgggttccgttaataaaagaagcagaacaaatcgcgtggttgcaacgtaaattgggcaatgcggcgcgcgttgaagatgtgcatcccatatcggaacggccacagtatttttctggtgatggtaaaagtggaaagatccaaacggtttgctttgaaggtgtgctcaccatcaacgacgcgccagcgttaatagatcttgtacagcaaggtattgggccagctaaatcgatgggatgtggcttgctatctttggctccactgtga

SEQ ID NO: 65 - DNA, 2667 bp, Escherichia coli
atggaaccttttaaatatatatgccattactggggaaaatcctcaaaaagcttgacgaaaggaaatgatattcatctgttaatttatcattgccttgatgttgctgctgttgcagattgctggtgggatcaatcagtcgtactgcaaaatactttttgccgaaatgaaatgctatcaaaacagagggtgaaggcctggctgttatttttcattgctcttcatgatattggaaagtttgatatacgattccaatataaatcagcagaaagttggctgaaattaaatcctgcaacgccatcacttaatggtccatcaacacaaatgtgccgtaaatttaatcatggtgcagccggtctgtattggtttaaccaggattcactttcagagcaatctctcggggattttttcagtttttttgatgccgctcctcatccttatgagtcctggtttccatgggtagaggccgttacaggacatcatggttttatattacattcccaggatcaagataagtcgcgttgggaaatgccagcttctctggcatcttatgctgcgcaagataaacaggctcgtgaggagtggatatctgtactggaagcattatttttaacgccagcggggttatctataaacgatataccacctgattgttcatcactgttagcaggtttttgctcgcttgctgactggttaggctcctggactacaacgaatacctttctgtttaatgaggatgcgccttccgacataaatgctctgagaacgtatttccaggaccgacagcaggatgcgagccgggtattggagttgagtggacttgtatcaaataagcgatgttatgaaggtgttcatgcactactggacaatggctatcaacccagacaattacaggtgttagttgatgctcttccagtagctcccgggctgacggtaatagaggcacctacaggctccggtaaaacggaaacagcgctggcctatgcttggaaacttattgatcaacaaattgcggatagtgttatttttgccctcccaacacaagctaccgcgaatgctatgcttacgagaatggaagcgagcgcgagccacttattttcatccccaaatcttattcttgctcatggcaattcacggtttaaccacctctttcaatcaataaaatcacgcgcgattactgaacaggggcaagaagaagcgtgggttcagtgttgtcagtggttgtcacaaagcaataagaaagtgtttcttgggcaaatcggcgtttgcacgattgatcaggtgttgatatcggtattgccagttaaacaccgctttatccgtggtttgggaattggtcgaagtgttttaattgttgatgaagttcatgcttacgacacctatatgaacggcttgctggaggcagtgctcaaggctcaggctgatgtgggagggagtgttattcttctttccgcaaccctaccaatgaaacaaaaacagaaacttctggatacttatggtctgcatacagatccagtggaaaataactccgcatatccactcattaactggcgaggtgtgaatggtgcgcaacgttttgatctgctagctcatccagaacaactcccgccccgcttttcgattcagccagaacctatttgtttagctgacatgttacctgaccttacgatgttagagcgaatgatcgcagcggcaaacgcgggtgcacaggtctgtcttatttgcaatttggttgacgttgcacaagtatgctaccaacggctaaaggagctaaataacacgcaagtagatatagatttgtttcatgcgcgctttacgctgaacgatcgtcgtgaaaaagagaatcgagttattagcaatttcggcaaaaatgggaagcgaaatgttggacggatacttgtcgcaacccaggtcgtggaacaatcactcgacgttgattttgattggttaattactcagcattgtcctgcagatttgcttttccaacgattgggccgtttacatcgccatcatcgcaaatatcgtcccgctggttttgagattcctgttgccaccattttgctgcctgatggcgagggttacggacgacatgagcatatttatagcaacgttagagtcatgtggcggacgcagcaacatattgaggagcttaatggagcatccttatttttccctgatgcttaccggcaatggctggatagcatttacgatgatgcggaaatggatgagccagaatgggtcggcaatggcatggataaatttgaaagcgccgagtgtgaaaaaaggttcaaggctcgcaaggtcctgcagtgggctgaagaatatagcttgcaggataacgatgaaaccattcttgcggtaacgagggatggggaaatgagcctgccattattgccttatgtacaaacgtcttcaggtaaacaactgctcgatggccaggtctacgaggacctaagtcatgaacagcagtatgaggcgcttgcacttaatcgcgtcaatgtacccttcacctggaaacgtagtttttctgaagtagtagatgaagatgggttactttggctggaagggaaacagaatctggatggatgggtctggcagggtaacagtattgttattacctatacaggggatgaagggatgaccagagtcatccctgcaaatcccaaataa

SEQ ID NO: 66 - DNA, 4107 bp, Streptococcus pyogenes
atggataagaaatactcaataggcttagatatcggcacaaatagcgtcggatgggcggtgatcactgatgaatataaggttccgtctaaaaagttcaaggttctgggaaatacagaccgccacagtatcaaaaaaaatcttataggggctcttttatttgacagtggagagacagcggaagcgactcgtctcaaacggacagctcgtagaaggtatacacgtcggaagaatcgtatttgttatctacaggagattttttcaaatgagatggcgaaagtagatgatagtttctttcatcgacttgaagagtcttttttggtggaagaagacaagaagcatgaacgtcatcctatttttggaaatatagtagatgaagttgcttatcatgagaaatatccaactatctatcatctgcgaaaaaaattggtagattctactgataaagcggatttgcgcttaatctatttggccttagcgcatatgattaagtttcgtggtcattttttgattgagggagatttaaatcctgataatagtgatgtggacaaactatttatccagttggtacaaacctacaatcaattatttgaagaaaaccctattaacgcaagtggagtagatgctaaagcgattctttctgcacgattgagtaaatcaagacgattagaaaatctcattgctcagctccccggtgagaagaaaaatggcttatttgggaatctcattgctttgtcattgggtttgacccctaattttaaatcaaattttgatttggcagaagatgctaaattacagctttcaaaagatacttacgatgatgatttagataatttattggcgcaaattggagatcaatatgctgatttgtttttggcagctaagaatttatcagatgctattttactttcagatatcctaagagtaaatactgaaataactaaggctcccctatcagcttcaatgattaaacgctacgatgaacatcatcaagacttgactcttttaaaagctttagttcgacaacaacttccagaaaagtataaagaaatcttttttgatcaatcaaaaaacggatatgcaggttatattgatgggggagctagccaagaagaattttataaatttatcaaaccaattttagaaaaaatggatggtactgaggaattattggtgaaactaaatcgtgaagatttgctgcgcaagcaacggacctttgacaacggctctattccccatcaaattcacttgggtgagctgcatgctattttgagaagacaagaagacttttatccatttttaaaagacaatcgtgagaagattgaaaaaatcttgacttttcgaattccttattatgttggtccattggcgcgtggcaatagtcgttttgcatggatgactcggaagtctgaagaaacaattaccccatggaattttgaagaagttgtcgataaaggtgcttcagctcaatcatttattgaacgcatgacaaactttgataaaaatcttccaaatgaaaaagtactaccaaaacatagtttgctttatgagtattttacggtttataacgaattgacaaaggtcaaatatgttactgaaggaatgcgaaaaccagcatttctttcaggtgaacagaagaaagccattgttgatttactcttcaaaacaaatcgaaaagtaaccgttaagcaattaaaagaagattatttcaaaaaaatagaatgttttgatagtgttgaaatttcaggagttgaagatagatttaatgcttcattaggtacctaccatgatttgctaaaaattattaaagataaagattttttggataatgaagaaaatgaagatatcttagaggatattgttttaacattgaccttatttgaagatagggagatgattgaggaaagacttaaaacatatgctcacctctttgatgataaggtgatgaaacagcttaaacgtcgccgttatactggttggggacgtttgtctcgaaaattgattaatggtattagggataagcaatctggcaaaacaatattagattttttgaaatcagatggttttgccaatcgcaattttatgcagctgatccatgatgatagtttgacatttaaagaagacattcaaaaagcacaagtgtctggacaaggcgatagtttacatgaacatattgcaaatttagctggtagccctgctattaaaaaaggtattttacagactgtaaaagttgttgatgaattggtcaaagtaatggggcggcataagccagaaaatatcgttattgaaatggcacgtgaaaatcagacaactcaaaagggccagaaaaattcgcgagagcgtatgaaacgaatcgaagaaggtatcaaagaattaggaagtcagattcttaaagagcatcctgttgaaaatactcaattgcaaaatgaaaagctctatctctattatctccaaaatggaagagacatgtatgtggaccaagaattagatattaatcgtttaagtgattatgatgtcgatcacattgttccacaaagtttccttaaagacgattcaatagacaataaggtcttaacgcgttctgataaaaatcgtggtaaatcggataacgttccaagtgaagaagtagtcaaaaagatgaaaaactattggagacaacttctaaacgccaagttaatcactcaacgtaagtttgataatttaacgaaagctgaacgtggaggtttgagtgaacttgataaagctggttttatcaaacgccaattggttgaaactcgccaaatcactaagcatgtggcacaaattttggatagtcgcatgaatactaaatacgatgaaaatgataaacttattcgagaggttaaagtgattaccttaaaatctaaattagtttctgacttccgaaaagatttccaattctataaagtacgtgagattaacaattaccatcatgcccatgatgcgtatctaaatgccgtcgttggaactgctttgattaagaaatatccaaaacttgaatcggagtttgtctatggtgattataaagtttatgatgttcgtaaaatgattgctaagtctgagcaagaaataggcaaagcaaccgcaaaatatttcttttactctaatatcatgaacttcttcaaaacagaaattacacttgcaaatggagagattcgcaaacgccctctaatcgaaactaatggggaaactggagaaattgtctgggataaagggcgagattttgccacagtgcgcaaagtattgtccatgccccaagtcaatattgtcaagaaaacagaagtacagacaggcggattctccaaggagtcaattttaccaaaaagaaattcggacaagcttattgctcgtaaaaaagactgggatccaaaaaaatatggtggttttgatagtccaacggtagcttattcagtcctagtggttgctaaggtggaaaaagggaaatcgaagaagttaaaatccgttaaagagttactagggatcacaattatggaaagaagttcctttgaaaaaaatccgattgactttttagaagctaaaggatataaggaagttaaaaaagacttaatcattaaactacctaaatatagtctttttgagttagaaaacggtcgtaaacggatgctggctagtgccggagaattacaaaaaggaaatgagctggctctgccaagcaaatatgtgaattttttatatttagctagtcattatgaaaagttgaagggtagtccagaagataacgaacaaaaacaattgtttgtggagcagcataagcattatttagatgagattattgagcaaatcagtgaattttctaagcgtgttattttagcagatgccaatttagataaagttcttagtgcatataacaaacatagagacaaaccaatacgtgaacaagcagaaaatattattcatttatttacgttgacgaatcttggagctcccgctgcttttaaatattttgatacaacaattgatcgtaaacgatatacgtctacaaaagaagttttagatgccactcttatccatcaatccatcactggtctttatgaaacacgcattgatttgagtcagctaggaggtgactga

SEQ ID NO: 67 - protein, 502 aa, Escherichia coli
MNLLIDNWIPVRPRNGGKVQIINLQSLYCSRDQWRLSLPRDDMELAALALLVCIGQIIAPAKDDVEFRHRIMNPLTEDEFQQLIAPWIDMFYLNHAEHPFMQTKGVKANDVTPMEKLLAGVSGATNCAFVNQPGQGEALCGGCTAIALFNQANQAPGFGGGFKSGLRGGTPVTTFVRGIDLRSTVLLNVLTLPRLQKQFPNESHTENQPTWIKPIKSNESIPASSIGFVRGLFWQPAHIELCDPIGIGKCSCCGQESNLRYTGFLKEKFTFTVNGLWPHPHSPCLVTVKKGEVEEKFLAFTTSAPSWTQISRVVVDKIIQNENGNRVAAVVNQFRNIAPQSPLELIMGGYRNNQASILERRHDVLMFNQGWQQYGNVINEIVTVGLGYKTALRKALYTFAEGFKNKDFKGAGVSVHETAERHFYRQSELLIPDVLANVNFSQADEVIADLRDKLHQLCEMLFNQSVAPYAHHPKLISTLALARATLYKHLRELKPQGGPSNG

SEQ ID NO: 68 - protein, 160 aa, Escherichia coli
MADEIDAMALYRAWQQLDNGSCAQIRRVSEPDELRDIPAFYRLVQPFGWENPRHQQALLRMVFCLSAGKNVIRHQDKKSEQTTGISLGRALANSGRINERRIFQLIRADRTADMVQLRRLLTHAEPVLDWPLMARMLTWWGKRERQQLLEDFVLTTNKNA

SEQ ID NO: 69 - protein, 363 aa, Escherichia coli
MSNFINIHVLISHSPSCLNRDDMNMQKDAIFGGKRRVRISSQSLKRAMRKSGYYAQNIGESSLRTIHLAQLRDVLRQKLGERFDQKIIDKTLALLSGKSVDEAEKISADAVTPWVVGEIAWFCEQVAKAEADNLDDKKLLKVLKEDIAAIRVNLQQGVDIALSGRMATSGMMTELGKVDGAMSIAHAITTHQVDSDIDWFTAVDDLQEQGSAHLGTQEFSSGVFYRYANINLAQLQENLGGASREQALEIATHVVHMLATEVPGAKQRTYAAFNPADMVMVNFSDMPLSMANAFEKAVKAKDGFLQPSIQAFNQYWDRVANGYGLNGAAAQFSLSDVDPITAQVKQMPTLEQLKSWVRNNGEA

SEQ ID NO: 70 - protein, 224 aa, Escherichia coli
MRSYLILRLAGPMQAWGQPTFEGTRPTGRFPTRSGLLGLLGACLGIQRDDTSSLQALSESVQFAVRCDELILDDRRVSVTGLRDYHTVLGAREDYRGLKSHETIQTWREYLCDASFTVALWLTPHATMVISELEKAVLKPRYTPYLGRRSCPLTHPLFLGTCQASDPQKALLNYEPVGGDIYSEESVTGHHLKFTARDEPMITLPRQFASREWYVIKGGMDVSQ

SEQ ID NO: 71 - protein, 199 aa, Escherichia coli
MYLSKVIIARAWSRDLYQLHQGLWHLFPNRPDAARDFLFHVEKRNTPEGCHVLLQSAQMPVSTAVATVIKTKQVEFQLQVGVPLYFRLRANPIKTILDNQKRLDSKGNIKRCRVPLIKEAEQIAWLQRKLGNAARVEDVHPISERPQYFSGDGKSGKIQTVCFEGVLTINDAPALIDLVQQGIGPAKSMGCGLLSLAPL

SEQ ID NO: 72 - protein, 888 aa, Escherichia coli
MEPFKYICHYWGKSSKSLTKGNDIHLLIYHCLDVAAVADCWWDQSVVLQNTFCRNEMLSKQRVKAWLLFFIALHDIGKFDIRFQYKSAESWLKLNPATPSLNGPSTQMCRKFNHGAAGLYWFNQDSLSEQSLGDFFSFFDAAPHPYESWFPWVEAVTGHHGFILHSQDQDKSRWEMPASLASYAAQDKQAREEWISVLEALFLTPAGLSINDIPPDCSSLLAGFCSLADWLGSWTTTNTFLFNEDAPSDINALRTYFQDRQQDASRVLELSGLVSNKRCYEGVHALLDNGYQPRQLQVLVDALPVAPGLTVIEAPTGSGKTETALAYAWKLIDQQIADSVIFALPTQATANAMLTRMEASASHLFSSPNLILAHGNSRFNHLFQSIKSRAITEQGQEEAWVQCCQWLSQSNKKVFLGQIGVCTIDQVLISVLPVKHRFIRGLGIGRSVLIVDEVHAYDTYMNGLLEAVLKAQADVGGSVILLSATLPMKQKQKLLDTYGLHTDPVENNSAYPLINWRGVNGAQRFDLLAHPEQLPPRFSIQPEPICLADMLPDLTMLERMIAAANAGAQVCLICNLVDVAQVCYQRLKELNNTQVDIDLFHARFTLNDRREKENRVISNFGKNGKRNVGRILVATQVVEQSLDVDFDWLITQHCPADLLFQRLGRLHRHHRKYRPAGFEIPVATILLPDGEGYGRHEHIYSNVRVMWRTQQHIEELNGASLFFPDAYRQWLDSIYDDAEMDEPEWVGNGMDKFESAECEKRFKARKVLQWAEEYSLQDNDETILAVTRDGEMSLPLLPYVQTSSGKQLLDGQVYEDLSHEQQYEALALNRVNVPFTWKRSFSEVVDEDGLLWLEGKQNLDGWVWQGNSIVITYTGDEGMTRVIPANPK

SEQ ID NO: 73 - protein, 1368 aa, Streptococcus pyogenes [sequence omitted]

SEQ ID NO: 74 - protein, 270 aa, Klebsiella pneumoniae
MELPNIMHPVAKLSTALAAALMLSGCMPGEIRPTIGQQMETGDQRFGDLVFRQLAPNVWQHTSYLDMPGFGAVASNGLIVRDGGRVLVVDTAWTDDQTAQILNWIKQEINLPVALAVVTHAHQDKMGGMDALHAAGIATYANALSNQLAPQEGMVAAQHSLTFAANGWVEPATAPNFGPLKVFYPGPGHTSDNITVGIDGTDIAFGGCLIKDSKAKSLGNLGDADTEHYAASARAFGAAFPKASMIVMSHSAPDSRAAITHTARMADKLR

SEQ ID NO: 75 - DNA, 813 bp, Klebsiella pneumoniae
atggaattgcccaatattatgcacccggtcgcgaagctgagcaccgcattagccgctgcattgatgctgagcgggtgcatgcccggtgaaatccgcccgacgattggccagcaaatggaaactggcgaccaacggtttggcgatctggttttccgccagctcgcaccgaatgtctggcagcacacttcctatctcgacatgccgggtttcggggcagtcgcttccaacggtttgatcgtcagggatggcggccgcgtgctggtggtcgataccgcctggaccgatgaccagaccgcccagatcctcaactggatcaagcaggagatcaacctgccggtcgcgctggcggtggtgactcacgcgcatcaggacaagatgggcggtatggacgcgctgcatgcggcggggattgcgacttatgccaatgcgttgtcgaaccagcttgccccgcaagaggggatggttgcggcgcaacacagcctgactttcgccgccaatggctgggtcgaaccagcaaccgcgcccaactttggcccgctcaaggtattttaccccggccccggccacaccagtgacaatatcaccgttgggatcgacggcaccgacatcgcttttggtggctgcctgatcaaggacagcaaggccaagtcgctcggcaatctcggtgatgccgacactgagcactacgccgcgtcagcgcgcgcgtttggtgcggcgttccccaaggccagcatgatcgtgatgagccattccgcccccgatagccgcgccgcaatcactcatacggcccgcatggccgacaagctgcgctga

SEQ ID NO: 76 - protein, 291 aa, Escherichia coli
MVKKSLRQFTLMATATVTLLLGSVPLYAQTADVQQKLAELERQSGGRLGVALINTADNSQILYRADERFAMCSTSKVMAAAAVLKKSESEPNLLNQRVEIKKSDLVNYNPIAEKHVNGTMSLAELSAAALQYSDNVAMNKLIAHVGGPASVTAFARQLGDETFRLDRTEPTLNTAIPGDPRDTTSPRAMAQTLRNLTLGKALGDSQRAQLVTWMKGNTTGAASIQAGLPASWVVGDKTGSGGYGTTNDIAVIWPKDRAPLILVTYFTQPQPKAESRRDVLASAAKIVTDGL

SEQ ID NO: 77 - DNA, 876 bp, Escherichia coli
atggttaaaaaatcactgcgccagttcacgctgatggcgacggcaaccgtcacgctgttgttaggaagtgtgccgctgtatgcgcaaacggcggacgtacagcaaaaacttgccgaattagagcggcagtcgggaggcagactgggtgtggcattgattaacacagcagataattcgcaaatactttatcgtgctgatgagcgctttgcgatgtgcagcaccagtaaagtgatggccgcggccgcggtgctgaagaaaagtgaaagcgaaccgaatctgttaaatcagcgagttgagatcaaaaaatctgaccttgttaactataatccgattgcggaaaagcacgtcaatgggacgatgtcactggctgagcttagcgcggccgcgctacagtacagcgataacgtggcgatgaataagctgattgctcacgttggcggcccggctagcgtcaccgcgttcgcccgacagctgggagacgaaacgttccgtctcgaccgtaccgagccgacgttaaacaccgccattccgggcgatccgcgtgataccacttcacctcgggcaatggcgcaaactctgcggaatctgacgctgggtaaagcattgggcgacagccaacgggcgcagctggtgacatggatgaaaggcaataccaccggtgcagcgagcattcaggctggactgcctgcttcctgggttgtgggggataaaaccggcagcggtggctatggcaccaccaacgatatcgcggtgatctggccaaaagatcgtgcgccgctgattctggtcacttacttcacccagcctcaacctaaggcagaaagccgtcgcgatgtattagcgtcggcggctaaaatcgtcaccgacggtttgtaa